European Patent Application EP 4 438 049 A1, published October 2, 2024. Title: 一种经遗传修饰的微生物及其应用. Applicant: 和度生物技术（上海）有限公司. Application CN. The sequence listing filed with the application follows.

SEQUENCE LISTING (243 sequences)

SEQ ID NO: 1 - protein, 317 aa, Akkermansia muciniphila
MSNWITDNKPAAMVAGVGLLLFLGLSATGYIVNSKRSELDKKISIAAKEIKSANAAEITPSRSSNEELEKELNRYAKAVGSLETAYKPFLASSALVPTTPTAFQNELKTFRDSLISSCKKKNILITDTSSWLGFQVYSTQAPSVQAASTLGFELKAINSLVNKLAECGLSKFIKVYRPQLPIETPANNPEESDEADQAPWTPMPLEIAFQGDRESVLKAMNAITGMQDYLFTVNSIRIRNERMMPPPIANPAAAKPAAAQPATGAASLTPADEAAAPAAPAIQQVIKPYMGKEQVFVQVSLNLVHFNQPKAQEPSED

SEQ ID NO: 2 - protein, 25 aa, Akkermansia muciniphila
AINSLVNKLAECGLSKFIKVYRPQL

SEQ ID NO: 3 - protein, 237 aa, Akkermansia muciniphila
SLETAYKPFLASSALVPTTPTAFQNELKTFRDSLISSCKKKNILITDTSSWLGFQVYSTQAPSVQAASTLGFELKAINSLVNKLAECGLSKFIKVYRPQLPIETPANNPEESDEADQAPWTPMPLEIAFQGDRESVLKAMNAITGMQDYLFTVNSIRIRNERMMPPPIANPAAAKPAAAQPATGAASLTPADEAAAPAAPAIQQVIKPYMGKEQVFVQVSLNLVHFNQPKAQEPSED

SEQ ID NO: 4 - DNA, 864 bp, Akkermansia muciniphila
  source 1..864: mol_type = genomic DNA
attgttaacagcaagcgtagcgagctggataagaaaatcagcattgcggcgaaagagatcaagagcgcgaacgcggcggaaattaccccgagccgtagcagcaacgaggaactggagaaagaactgaaccgttacgcgaaggcggttggtagcctggaaaccgcgtataaaccgtttctggcgagcagcgcgctggtgccgaccaccccgaccgcgttccaaaacgagctgaaaacctttcgtgacagcctgatcagcagctgcaagaaaaagaacatcctgattaccgataccagcagctggctgggcttccaggtttacagcacccaagcgccgagcgtgcaggcggcgagcaccctgggttttgagctgaaagcgattaacagcctggttaacaagctggcggaatgcggcctgagcaaattcatcaaggtgtatcgtccgcagctgccgattgaaaccccggcgaacaacccggaggaaagcgacgaagcggatcaggcgccgtggaccccgatgccgctggagatcgcgttccagggtgaccgtgaaagcgttctgaaagcgatgaacgcgattaccggcatgcaagattacctgtttaccgtgaacagcatccgtattcgtaacgaacgtatgatgccgccgccaatcgcgaacccggctgcggcgaagccggctgcggcgcagccggcgaccggtgcggcgagcctgaccccggcggacgaggctgcggcgccggctgcgccggcgatccagcaagttattaaaccgtatatgggcaaggaacaggtgttcgttcaagtgagcctgaacctggtgcactttaaccagccgaaagcgcaagagccgagcgaagattga

SEQ ID NO: 5 - protein, 287 aa, Akkermansia muciniphila
IVNSKRSELDKKISIAAKEIKSANAAEITPSRSSNEELEKELNRYAKAVGSLETAYKPFLASSALVPTTPTAFQNELKTFRDSLISSCKKKNILITDTSSWLGFQVYSTQAPSVQAASTLGFELKAINSLVNKLAECGLSKFIKVYRPQLPIETPANNPEESDEADQAPWTPMPLEIAFQGDRESVLKAMNAITGMQDYLFTVNSIRIRNERMMPPPIANPAAAKPAAAQPATGAASLTPADEAAAPAAPAIQQVIKPYMGKEQVFVQVSLNLVHFNQPKAQEPSED

SEQ ID NO: 6 - DNA, 861 bp, synthetic construct
  source 1..861: mol_type = other DNA
attgttaacagcaagcgtagcgagctggataagaaaatcagcattgcggcgaaagagatcaagagcgcgaacgcggcggaaattaccccgagccgtagcagcaacgaggaactggagaaagaactgaaccgttacgcgaaggcggttggtagcctggaaaccgcgtataaaccgtttctggcgagcagcgcgctggtgccgaccaccccgaccgcgttccaaaacgagctgaaaacctttcgtgacagcctgatcagcagctgcaagaaaaagaacatcctgattaccgataccagcagctggctgggcttccaggtttacagcacccaagcgccgagcgtgcaggcggcgagcaccctgggttttgagctgaaagcgattaacagcctggttaacaagctggcggaatgcggcctgagcaaattcatcaaggtgtatcgtccgcagctgccgattgaaaccccggcgaacaacccggaggaaagcgacgaagcggatcaggcgccgtggaccccgatgccgctggagatcgcgttccagggtgaccgtgaaagcgttctgaaagcgatgaacgcgattaccggcatgcaagattacctgtttaccgtgaacagcatccgtattcgtaacgaacgtatgatgccgccgccaatcgcgaacccggctgcggcgaagccggctgcggcgcagccggcgaccggtgcggcgagcctgaccccggcggacgaggctgcggcgccggctgcgccggcgatccagcaagttattaaaccggctatgggcaaggaacaggtgttcgttcaagtgagcctgaacctggtgcactttaaccagccgaaagcgcaagagccgagcgaagat

SEQ ID NO: 7 - protein, 287 aa, synthetic construct
IVNSKRSELDKKISIAAKEIKSANAAEITPSRSSNEELEKELNRYAKAVGSLETAYKPFLASSALVPTTPTAFQNELKTFRDSLISSCKKKNILITDTSSWLGFQVYSTQAPSVQAASTLGFELKAINSLVNKLAECGLSKFIKVYRPQLPIETPANNPEESDEADQAPWTPMPLEIAFQGDRESVLKAMNAITGMQDYLFTVNSIRIRNERMMPPPIANPAAAKPAAAQPATGAASLTPADEAAAPAAPAIQQVIKPAMGKEQVFVQVSLNLVHFNQPKAQEPSED

SEQ ID NO: 8 - DNA, 861 bp, synthetic construct
  source 1..861: mol_type = other DNA
attgttaacagcaagcgtagcgagctggataagaaaatcagcattgcggcgaaagagatcaagagcgcgaacgcggcggaaattaccccgagccgtagcagcaacgaggaactggagaaagaactgaaccgttacgcgaaggcggttggtagcctggaaaccgcgtataaaccgtttctggcgagcagcgcgctggtgccgaccaccccgaccgcgttccaaaacgagctgaaaacctttcgtgacagcctgatcagcagctgcaagaaaaagaacatcctgattaccgataccagcagctggctgggcttccaggtttacagcacccaagcgccgagcgtgcaggcggcgagcaccctgggttttgagctgaaagcgattaacagcctggttaacaagctggcggaatgcggcctgagcaaattcatcaaggtgtatcgtccgcagctgccgattgaaaccccggcgaacaacccggaggaaagcgacgaagcggatcaggcgccgtggaccccgatgccgctggagatcgcgttccagggtgaccgtgaaagcgttctgaaagcgatgaacgcgattaccggcatgcaagattacctgtttaccgtgaacagcatccgtattcgtaacgaacgtatgatgccgccgccaatcgcgaacccggctgcggcgaagccggctgcggcgcagccggcgaccggtgcggcgagcctgaccccggcggacgaggctgcggcgccggctgcgccggcgatccagcaagttattaaaccgagcatgggcaaggaacaggtgttcgttcaagtgagcctgaacctggtgcactttaaccagccgaaagcgcaagagccgagcgaagat

SEQ ID NO: 9 - protein, 287 aa, synthetic construct
IVNSKRSELDKKISIAAKEIKSANAAEITPSRSSNEELEKELNRYAKAVGSLETAYKPFLASSALVPTTPTAFQNELKTFRDSLISSCKKKNILITDTSSWLGFQVYSTQAPSVQAASTLGFELKAINSLVNKLAECGLSKFIKVYRPQLPIETPANNPEESDEADQAPWTPMPLEIAFQGDRESVLKAMNAITGMQDYLFTVNSIRIRNERMMPPPIANPAAAKPAAAQPATGAASLTPADEAAAPAAPAIQQVIKPSMGKEQVFVQVSLNLVHFNQPKAQEPSED

SEQ ID NO: 10 - DNA, 483 bp, Homo sapiens
  source 1..483: mol_type = genomic DNA
agcccgggtcagggtacccaaagcgaaaacagctgcacccacttcccgggcaacctgccgaacatgctgcgtgacctgcgtgatgcgttcagccgtgtgaaaaccttcttccagatgaaagaccaactggataacctgctgctgaaggagagcctgctggaggacttcaaaggttacctgggctgccaggcgctgagcgaaatgatccaattttatctggaggaagtgatgccgcaggcggagaaccaagacccggatattaaggcgcacgttaacagcctgggcgagaacctgaaaaccctgcgtctgcgtctgcgtcgttgccaccgtttcctgccgtgcgagaacaaaagcaaggcggtggaacaggttaagaacgcgtttaacaaactgcaagagaagggcatctataaagcgatgagcgaattcgatatctttattaactacatcgaggcgtatatgaccatgaaaattcgtaactag

SEQ ID NO: 11 - protein, 160 aa, Homo sapiens
SPGQGTQSENSCTHFPGNLPNMLRDLRDAFSRVKTFFQMKDQLDNLLLKESLLEDFKGYLGCQALSEMIQFYLEEVMPQAENQDPDIKAHVNSLGENLKTLRLRLRRCHRFLPCENKSKAVEQVKNAFNKLQEKGIYKAMSEFDIFINYIEAYMTMKIRN

SEQ ID NO: 12 - DNA, 481 bp, synthetic construct
  source 1..481: mol_type = other DNA
agcgcgggtcagggtacccaaagcgaaaacagctgcacccacttcccgggcaacctgccgaacatgctgcgtgacctgcgtgatgcgttcagccgtgtgaaaaccttcttccagatgaaagaccaactggataacctgctgctgaaggagagcctgctggaggacttcaaaggttacctgggctgccaggcgctgagcgaaatgatccaattttatctggaggaagtgatgccgcaggcggagaaccaagacccggatattaaggcgcacgttaacagcctgggcgagaacctgaaaaccctgcgtctgcgtctgcgtcgttgccaccgtttcctgccgtgcgagaacaaaagcaaggcggtggaacaggttaagaacgcgtttaacaaactgcaagagaagggcatctataaagcgatgagcgaattcgatatctttattaactacatcgaggcgtatatgaccatgaaaattcgtaact

SEQ ID NO: 13 - protein, 160 aa, synthetic construct
SAGQGTQSENSCTHFPGNLPNMLRDLRDAFSRVKTFFQMKDQLDNLLLKESLLEDFKGYLGCQALSEMIQFYLEEVMPQAENQDPDIKAHVNSLGENLKTLRLRLRRCHRFLPCENKSKAVEQVKNAFNKLQEKGIYKAMSEFDIFINYIEAYMTMKIRN

SEQ ID NO: 14 - DNA, 441 bp, Homo sapiens
  source 1..441: mol_type = genomic DNA
gcgccgatcagcagccactgccgtctggacaaaagcaacttccagcaaccgtatattaccaaccgtacctttatgctggcgaaagaggcgagcctggcggacaacaacaccgatgtgcgtctgatcggcgagaaactgttccacggcgttagcatgagcgaacgttgctacctgatgaagcaggtgctgaactttaccctggaggaagttctgttcccgcaaagcgatcgttttcagccgtatatgcaagaggtggttccgttcctggcgcgtctgagcaaccgtctgagcacctgccacatcgaaggtgacgatctgcacattcagcgtaacgtgcaaaaactgaaggacaccgttaaaaagctgggcgagagcggcgaaatcaaagcgattggcgaactggatctgctgtttatgagcctgcgtaacgcgtgcatttag

SEQ ID NO: 15 - protein, 146 aa, Homo sapiens
APISSHCRLDKSNFQQPYITNRTFMLAKEASLADNNTDVRLIGEKLFHGVSMSERCYLMKQVLNFTLEEVLFPQSDRFQPYMQEVVPFLARLSNRLSTCHIEGDDLHIQRNVQKLKDTVKKLGESGEIKAIGELDLLFMSLRNACI

SEQ ID NO: 16 - DNA, 35 bp, synthetic construct
  source 1..35: mol_type = other DNA
ttgacagctagctcagtcctaggtataatgctagc

SEQ ID NO: 17 - DNA, 35 bp, synthetic construct
  source 1..35: mol_type = other DNA
tttacagctagctcagtcctaggtattatgctagc

SEQ ID NO: 18 - DNA, 35 bp, synthetic construct
  source 1..35: mol_type = other DNA
ttgacagctagctcagtcctaggtactgtgctagc

SEQ ID NO: 19 - DNA, 35 bp, synthetic construct
  source 1..35: mol_type = other DNA
ctgatagctagctcagtcctagggattatgctagc

SEQ ID NO: 20 - DNA, 35 bp, synthetic construct
  source 1..35: mol_type = other DNA
tttacagctagctcagtcctagggactgtgctagc

SEQ ID NO: 21 - DNA, 35 bp, synthetic construct
  source 1..35: mol_type = other DNA
tttacggctagctcagtcctaggtacaatgctagc

SEQ ID NO: 22 - DNA, 35 bp, synthetic construct
  source 1..35: mol_type = other DNA
tttatggctagctcagtcctaggtacaatgctagc

SEQ ID NO: 23 - DNA, 35 bp, synthetic construct
  source 1..35: mol_type = other DNA
ttgacagctagctcagtcctagggattgtgctagc

SEQ ID NO: 24 - DNA, 77 bp, synthetic construct
  source 1..77: mol_type = other DNA
aaagtgttttgtaatcataaagaaatattaaggtggggtaggaatagtataatatgtttattcaaccgaacttaatg

SEQ ID NO: 25 - DNA, 176 bp, synthetic construct
  source 1..176: mol_type = other DNA
gggccgagcatgtggaaacacctctgccaggtcaagcccgcagccatgccgcatgtttttttcttgaccgcccgggcagaaccgtcgggcggagccgtgtcatgctccacacacgctacatggaaagaaacaagagatttttgctagccacagttcggtttttggtgtaactaatc

SEQ ID NO: 26 - DNA, 339 bp, synthetic construct
  source 1..339: mol_type = other DNA
gtaaatttaggattaatcctggaactttttttgtcgcccagccaatgctttcagtcgtgactaattttccttgcggaggcttgtctgaagcggtttccgcgattttcttctgtaaattgtcgctgacaaaaaagattaaacgtaccttatacaagacttttttttcatatgcctgacggagttcacacttgtaagttttcaactacgttgtagactttacatcgccaggggtgctcggcataagccgaagatatcggtagagttaatattgagcagatccccggtgaaggatttaaccgtgttatctcgttggagatattcatggcgtattttggatga

SEQ ID NO: 27 - DNA, 35 bp, synthetic construct
  source 1..35: mol_type = other DNA
ttgacggctagctcagtcctaggtacagtgctagc

SEQ ID NO: 28 - DNA, 35 bp, synthetic construct
  source 1..35: mol_type = other DNA
ttgacagctagctcagtcctaggtattgtgctagc

SEQ ID NO: 29 - DNA, 35 bp, synthetic construct
  source 1..35: mol_type = other DNA
tttacggctagctcagtcctaggtactatgctagc

SEQ ID NO: 30 - DNA, 35 bp, synthetic construct
  source 1..35: mol_type = other DNA
tttacggctagctcagtcctaggtatagtgctagc

SEQ ID NO: 31 - DNA, 35 bp, synthetic construct
  source 1..35: mol_type = other DNA
tttacggctagctcagccctaggtattatgctagc

SEQ ID NO: 32 - DNA, 35 bp, synthetic construct
  source 1..35: mol_type = other DNA
ctgacagctagctcagtcctaggtataatgctagc

SEQ ID NO: 33 - DNA, 35 bp, synthetic construct
  source 1..35: mol_type = other DNA
ttgacggctagctcagtcctaggtatagtgctagc

SEQ ID NO: 34 - DNA, 35 bp, synthetic construct; identical to SEQ ID NO: 19
  source 1..35: mol_type = other DNA

SEQ ID NO: 35 - DNA, 35 bp, synthetic construct
  source 1..35: mol_type = other DNA
ctgatggctagctcagtcctagggattatgctagc

SEQ ID NO: 36 - DNA, 35 bp, synthetic construct
  source 1..35: mol_type = other DNA
tttatagctagctcagcccttggtacaatgctagc

SEQ ID NO: 37 - DNA, 35 bp, synthetic construct
  source 1..35: mol_type = other DNA
ttgacagctagctcagtcctagggactatgctagc

SEQ ID NO: 38 - DNA, 35 bp, synthetic construct
  source 1..35: mol_type = other DNA
ttgacggctagctcagtcctaggtattgtgctagc

SEQ ID NO: 39 - DNA, 30 bp, synthetic construct
  source 1..30: mol_type = other DNA
ggtttcaaaattgtgatctatatttaacaa

SEQ ID NO: 40 - DNA, 30 bp, synthetic construct
  source 1..30: mol_type = other DNA
gtttatacataggcgagtactctgttatgg

SEQ ID NO: 41 - DNA, 30 bp, synthetic construct
  source 1..30: mol_type = other DNA
agaggttccaactttcaccataatgaaaca

SEQ ID NO: 42 - DNA, 30 bp, synthetic construct
  source 1..30: mol_type = other DNA
taaacaactaacggacaattctacctaaca

SEQ ID NO: 43 - DNA, 30 bp, synthetic construct
  source 1..30: mol_type = other DNA
ggctagctcagtcctaggtattatgctagc

SEQ ID NO: 44 - DNA, 30 bp, synthetic construct
  source 1..30: mol_type = other DNA
aaagtgtgacgccgtgcaaataatcaatgt

SEQ ID NO: 45 - DNA, 30 bp, synthetic construct
  source 1..30: mol_type = other DNA
ggctagctcagtcctaggtactatgctagc

SEQ ID NO: 46 - DNA, 30 bp, synthetic construct
  source 1..30: mol_type = other DNA
caccttcgggtgggcctttctgcgtttata

SEQ ID NO: 47 - DNA, 178 bp, synthetic construct
  source 1..178: mol_type = other DNA
aagctgttgtgaccgcttgctctagccagctatcgagttgtgaaccgatccatctagcaattggtctcgatctagcgataggcttcgatctagctatgtatcactcattaggcaccccaggctttacactttatgcttccggctcgtataatgtgtggtgctggttagcgcttgctat

SEQ ID NO: 48 - DNA, 190 bp, synthetic construct
  source 1..190: mol_type = other DNA
aagctgttgtgaccgcttgctctagccagctatcgagttgtgaaccgatccatctagcaattggtctcgatctagcgataggcttcgatctagctatgtagaaacgccgtgtgctcgatcgcttgataaggtccacgtagctgctataattgcttcaacagaacatattgactatccggtattacccggc

SEQ ID NO: 49 - DNA, 30 bp, synthetic construct
  source 1..30: mol_type = other DNA
catacgccgttatacgttgtttacgctttg

SEQ ID NO: 50 - DNA, 30 bp, synthetic construct
  source 1..30: mol_type = other DNA
atatatatatatatataatggaagcgtttt

SEQ ID NO: 51 - DNA, 30 bp, synthetic construct
  source 1..30: mol_type = other DNA
ccccgaaagcttaagaatataattgtaagc

SEQ ID NO: 52 - DNA, 30 bp, synthetic construct
  source 1..30: mol_type = other DNA
ggctagctcagtcctaggtacagtgctagc

SEQ ID NO: 53 - DNA, 30 bp, synthetic construct
  source 1..30: mol_type = other DNA
tgctagctactagagattaaagaggagaaa

SEQ ID NO: 54 - DNA, 52 bp, synthetic construct
  source 1..52: mol_type = other DNA
cccaggctttacactttatgcttccggctcgtataatgtgtggaattgtgag

SEQ ID NO: 55 - DNA, 44 bp, synthetic construct
  source 1..44: mol_type = other DNA
ttgacaattaatcatccggctcgtataatgtgtggaattgtgag

SEQ ID NO: 56 - DNA, 73 bp, synthetic construct
  source 1..73: mol_type = other DNA
taattcctaatttttgttgacactctatcgttgatagagttattttaccactccctatcagtgatagagaaaa

SEQ ID NO: 57 - DNA, 74 bp, synthetic construct
  source 1..74: mol_type = other DNA
tccctatcagtgatagagattgacatccctatcagtgatagagatactgagcacatcagcaggacgcactgacc

SEQ ID NO: 58 - DNA, 68 bp, synthetic construct
  source 1..68: mol_type = other DNA
attccactaatttattccatgtcacacttttcgcatctttgttatgctatggttatttcataccataa

SEQ ID NO: 59 - DNA, 76 bp, synthetic construct
  source 1..76: mol_type = other DNA
ataaatgtgagcggataacaattgacattgtgagcggataacaagatactgagcacatcagcaggacgcactgacc

SEQ ID NO: 60 - DNA, 65 bp, synthetic construct
  source 1..65: mol_type = other DNA
aaaaacgccgcaaagtttgagcgaagtcaataaactctctacccattcagggcaatatctctctt

SEQ ID NO: 61 - DNA, 99 bp, synthetic construct
  source 1..99: mol_type = other DNA
tgaataaatagtgcccgtaatatcagggaatgaccccacataaaatgtggcataaaagatgcatactgtagtcgagagcgcgtatgcgtgatttgatta

SEQ ID NO: 62 - DNA, 22 bp, synthetic construct
  source 1..22: mol_type = other DNA
ggaggaaaaattaaaaaagaac

SEQ ID NO: 63 - DNA, 12 bp, synthetic construct
  source 1..12: mol_type = other DNA
aaagaggagaaa

SEQ ID NO: 64-67 - skipped (4 entries)

SEQ ID NO: 68 - protein, 10 aa, synthetic construct
MRKGEEKEVN

SEQ ID NO: 69 - DNA, 33 bp, synthetic construct
  source 1..33: mol_type = other DNA
atgcgtaaaggcgaagagaaggaggttaactga

SEQ ID NO: 70 - protein, 17 aa, synthetic construct
MKAIFVLKHLNHAKEVF

SEQ ID NO: 71 - DNA, 54 bp, synthetic construct
  source 1..54: mol_type = other DNA
atgaaagcaattttcgtactgaaacatcttaatcatgctaaggaggttttctaa

SEQ ID NO: 72 - protein, 10 aa, synthetic construct
MIMSGYKEVN

SEQ ID NO: 73 - DNA, 33 bp, synthetic construct
  source 1..33: mol_type = other DNA
atgattatgtccggttataaggaggttaactga

SEQ ID NO: 74 - protein, 14 aa, synthetic construct
MKIEAGKLVQKEVN

SEQ ID NO: 75 - DNA, 45 bp, synthetic construct
  source 1..45: mol_type = other DNA
atgaaaatcgaagcaggtaaactggtacagaaggaggttaactga

SEQ ID NO: 76 - DNA, 72 bp, synthetic construct
  source 1..72: mol_type = other DNA
caaataaaacgaaaggctcagtcgaaagactgggcctttcgttttatctgttgtttgtcggtgaacgctctc

SEQ ID NO: 77 - DNA, 59 bp, synthetic construct
  source 1..59: mol_type = other DNA
caaataaaacgaaagactgggcctttcgttttatctgttgtttgtcggtgaacgctctc

SEQ ID NO: 78 - DNA, 28 bp, synthetic construct
  source 1..28: mol_type = other DNA
ggctcaccttcgggtgggcctttctgcg

SEQ ID NO: 79 - DNA, 66 bp, synthetic construct
  source 1..66: mol_type = other DNA
tagtacctgtgaagtgaaaaatggcgcacattgtgcgccattttttttgtctgccgtttaccgcta

SEQ ID NO: 80 - protein, 30 aa, synthetic construct
MSNWITDNKPAAMVAGVGLLLFLGLSATGY

SEQ ID NO: 81 - protein, 22 aa, synthetic construct
MEFFKKTALAALVMGFSGAALA

SEQ ID NO: 82 - protein, 23 aa, synthetic construct
MSIQHFRVALIPFFAAFCLPVFA

SEQ ID NO: 83 - protein, 31 aa, synthetic construct
MILNRLSTLGIITFGMLSFAPGPPPGPPRVS

SEQ ID NO: 84 - protein, 20 aa, synthetic construct
EGNTREDNFKHLLGNDNVKR

SEQ ID NO: 85 - protein, 21 aa, synthetic construct
MKKAKAIFLFILIVSGFLLVA

SEQ ID NO: 86 - protein, 19 aa, synthetic construct
MKKIWLALAGLVLAFSASA

SEQ ID NO: 87 - protein, 21 aa, synthetic construct
MNKVKFYVLFTALLSPLCAHG

SEQ ID NO: 88 - protein, 25 aa, synthetic construct
MKSLFKVTLLATTMAVALHAPITFA

SEQ ID NO: 89 - protein, 25 aa, synthetic construct
MMITLRKLPLAVAVAAGVMSAQAMA

SEQ ID NO: 90 - protein, 20 aa, synthetic construct
MKATKLVLGAVILGSTLLAG

SEQ ID NO: 91 - protein, 21 aa, synthetic construct
MNKVKCYVLFTALLSSLYAHG

SEQ ID NO: 92 - protein, 26 aa, synthetic construct
MKIKTGARILALSALTTMMFSASALA

SEQ ID NO: 93 - protein, 23 aa, synthetic construct
MNKKVLTLSAVMASMLFGAAAHA

SEQ ID NO: 94 - protein, 27 aa, synthetic construct
MGLGKKLSVAVAASFMSLTISLPGVQA

SEQ ID NO: 95 - protein, 21 aa, synthetic construct
MKKTAIAIAVALAGFATVAQA

SEQ ID NO: 96 - protein, 21 aa, synthetic construct
MKVKVLSLLVPALLVAGAANA

SEQ ID NO: 97 - protein, 22 aa, synthetic construct
MMKRNILAVIVPALLVAGTANA

SEQ ID NO: 98 - protein, 20 aa, synthetic construct
MRAKLLGIVLTTPIAISPFA

SEQ ID NO: 99 - protein, 28 aa, synthetic construct
MTMTRLKISKTLLAVMLTSAVATGSAYA

SEQ ID NO: 100 - protein, 22 aa, synthetic construct
MKYLLPTAAAGLLLLAAQPAMA

SEQ ID NO: 101 - protein, 26 aa, synthetic construct
MYSSSRKRCPKTKWALKLLTAAFLAA

SEQ ID NO: 102 - protein, 20 aa, synthetic construct
MLRNGNKYLLMLVSIIMLTA

SEQ ID NO: 103 - protein, 21 aa, synthetic construct
MKQSTIALALLPLLFTPVTKA

SEQ ID NO: 104 - protein, 21 aa, synthetic construct
MKKSTLALVVMGIVASASVQA

SEQ ID NO: 105 - protein, 49 aa, synthetic construct
MNKIYSLKYSAATGGLIAVSELAKRVSGKTNRKLVATMLSLAVAGTVNA

SEQ ID NO: 106 - protein, 23 aa, synthetic construct
MMTKIKLLMLIIFYLIISASAHA

SEQ ID NO: 107 - protein, 20 aa, synthetic construct
MKKWLLAAGLGLALATSAQA

SEQ ID NO: 108 - protein, 19 aa, synthetic construct
MKKLMLAIFISVLSFPSFS

SEQ ID NO: 109 - protein, 23 aa, synthetic construct
MKKNIAFLLASMFVFSIATNAYA

SEQ ID NO: 110 - protein, 20 aa, synthetic construct
MKNWKTLLLGIAMIANTSFA

SEQ ID NO: 111 - protein, 21 aa, synthetic construct
MKQALRVAFGFLILWASVLHA

SEQ ID NO: 112 - protein, 39 aa, synthetic construct
MNNNDLFQASRRRFLAQLGGLTVAGMLGPSLLTPRRATA

SEQ ID NO: 113 - protein, 18 aa, synthetic construct
MRVLLFLLLSLFMLPAFS

SEQ ID NO: 114 - protein, 27 aa, synthetic construct
MKKKIISAILMSTVILSAAAPLSGVYA

SEQ ID NO: 115 - protein, 28 aa, synthetic construct
MFKFKKKFLVGLTAAFMSISMFSATASA

SEQ ID NO: 116 - protein, 21 aa, synthetic construct
MKKRGAFLGLLLVSACASVFA

SEQ ID NO: 117 - protein, 43 aa, synthetic construct
MKLLKVAAIAAIVFSGSALAGVVPQYGGGGGNHGGGGNNSGPN

SEQ ID NO: 118 - protein, 42 aa, synthetic construct
VIKFLSALILLLVTTAAQAGVVPQYGGGGGNHGGGGNNSGPN

SEQ ID NO: 119 - protein, 46 aa, synthetic construct
MMTKIKLLMLIIFYLIISASAHAGVVPQYGGGGGNHGGGGNNSGPN

SEQ ID NO: 120 - protein, 50 aa, synthetic construct
MKKKIISAILMSTVILSAAAPLSGVYAGVVPQYGGGGGNHGGGGNNSGPN

SEQ ID NO: 121 - protein, 46 aa, synthetic construct
MSKRTFAVILTLLCSFCIGQALAGVVPQYGGGGGNHGGGGNNSGPN

SEQ ID NO: 122 - protein, 152 aa, synthetic construct
MKLLKVAAIAAIVFSGSALAGVVPQYGGGGGNHGGGGNNSGPNSELNIYQYGGGNSALALQADARNSDLTITQHGGGNGADVGQGSDDSSIDLTQRGFGNSATLDQWNGKDSTMTVKQFGGGNGAAVDQTASNSSVNVTQVGFGNNATAHQY

SEQ ID NO: 123 - DNA, 90 bp, synthetic construct
  source 1..90: mol_type = other DNA
atgagcaactggatcaccgacaacaaaccggctgcgatggttgcgggtgtgggcctgctgctgttcctgggtctgagcgcgaccggctac

SEQ ID NO: 124 - DNA, 60 bp, synthetic construct
  source 1..60: mol_type = other DNA
gaaggaaacactcgtgaagacaattttaaacatttattaggtaatgacaatgttaaacgc

SEQ ID NO: 125 - DNA, 57 bp, synthetic construct
  source 1..57: mol_type = other DNA
atgaagaaaatctggctggcgctggcgggtctggtgctggcgttcagcgcgagcgcg

SEQ ID NO: 126 - DNA, 63 bp, synthetic construct
  source 1..63: mol_type = other DNA
atgaagaaaaccgcgattgcgattgcggtggcgctggcgggtttcgcgaccgttgcgcaggcg

SEQ ID NO: 127 - DNA, 66 bp, synthetic construct
  source 1..66: mol_type = other DNA
atgaagtacctgctgccgaccgcggcggcgggtctgctgctgctggcggcgcagccggcgatggcg

SEQ ID NO: 128 - DNA, 147 bp, synthetic construct
  source 1..147: mol_type = other DNA
atgaataaaatatactcccttaaatatagtgctgccactggcggactcattgctgtttctgaattagcgaaaagagtttctggtaaaacaaaccgaaaacttgtagcaacaatgttgtctctggctgttgccggtacagtaaatgca

SEQ ID NO: 129 - DNA, 78 bp, synthetic construct
  source 1..78: mol_type = other DNA
aagaaaaagatcattagcgcgatcctgatgagcaccgtgattctgagcgcggcggcgccgctgagcggtgtttatgcg

SEQ ID NO: 130 - DNA, 129 bp, synthetic construct
  source 1..129: mol_type = other DNA
atgaaacttttaaaagtagcagcaattgcagcaatcgtattctccggtagcgctctggcaggtgttgttcctcagtacggcggcggcggtggcaaccacggtggtggcggtaataacagcggtccgaat

SEQ ID NO: 131 - DNA, 126 bp, synthetic construct
  source 1..126: mol_type = other DNA
gtgataaagtttctgtcagcactgatattacttcttgttaccaccgccgttcaggccggtgttgttcctcagtacggcggcggcggtggcaaccacggtggtggcggtaataacagcggtccgaat

SEQ ID NO: 132 - DNA, 138 bp, synthetic construct
  source 1..138: mol_type = other DNA
atgatgactaaaataaagttattgatgctcattatattttatttaatcatttcggccagcgcccatgctggtgttgttcctcagtacggcggcggcggtggcaaccacggtggtggcggtaataacagcggtccgaat

SEQ ID NO: 133 - DNA, 150 bp, synthetic construct
  source 1..150: mol_type = other DNA
atgaagaaaaagatcattagcgcgatcctgatgagcaccgtgattctgagcgcggcggcgccgctgagcggtgtttatgcgggtgttgttcctcagtacggcggcggcggtggcaaccacggtggtggcggtaataacagcggtccgaat

SEQ ID NO: 134 - DNA, 138 bp, synthetic construct
  source 1..138: mol_type = other DNA
atgtcaaaacgaacattcgcggtgatattaaccttgttgtgtagcttctgtattggccaggcgcttgcaggtgttgttcctcagtacggcggcggcggtggcaaccacggtggtggcggtaataacagcggtccgaat

SEQ ID NO: 135 - DNA, 456 bp, synthetic construct
  source 1..456: mol_type = other DNA
atgaaacttttaaaagtagcagcaattgcagcaatcgtattctccggtagcgctctggcaggtgttgttcctcagtacggcggcggcggtggcaaccacggtggtggcggtaataacagcggtccgaattcagagctgaatatttaccagtacggtggcggtaactctgctcttgctctgcaagctgacgcccgtaactctgatctgaccattacccagcacggcggcggtaatggcgcagatgtgggccaaggttctgatgacagctcaatcgatctgactcagcgtggtttcggcaacagcgctactcttgatcagtggaatggtaaagattctactatgactgttaaacagttcggtggcggtaacggtgctgctgttgaccagactgcatctaactccagcgttaacgtcactcaggttggctttggtaacaacgcgaccgctcatcagtac

SEQ ID NO: 136 - DNA, 15460 bp, synthetic construct
  source 1..15460: mol_type = other DNA
ctgctcgcgcaggctgggtgccaagctctcgggtaacatcaaggcccgatccttggagcccttgccctcccgcacgatgatcgtgccgtgatcgaaatccagatccttgacccgcagttgcaaaccctcactgatccgcatgcggatcttgctgtaggcataggcttggttatgccggtactgccgggcctcttgcgggattacgaaatcatcctgtggagcttagtaggtttagcaagatggcagcgcctaaatgtagaatgataaaaggattaagagattaatttccctaaaaatgataaaacaagcgttttgaaagcgcttgtttttttggtttgcagtcagagtagaatagaagtatcaaaaaaagcaccgactcggtgccactttttcaagttgataacggactagccttattttaacttgctatgctgttttgaatggttccaacaagattattttataacttttataacaaataatcaaggagaaattcaaagaaatttatcagccataaaacaatacttaatactatagaatgataacaaaataaactactttttaaaagaattttgtgttataatctatttattattaagtattgggtaatattttttgaagagatattttgaaaaagaaaaattaaagcatattaaactaatttcggaggtcattaaaactattattgaaatcatcaaactcattatggatttaatttaaactttttattttaggaggcaaaaatggataagaaatactcaataggcttagatatcggcacaaatagcgtcggatgggcggtgatcactgatgaatataaggttccgtctaaaaagttcaaggttctgggaaatacagaccgccacagtatcaaaaaaaatcttataggggctcttttatttgacagtggagagacagcggaagcgactcgtctcaaacggacagctcgtagaaggtatacacgtcggaagaatcgtatttgttatctacaggagattttttcaaatgagatggcgaaagtagatgatagtttctttcatcgacttgaagagtcttttttggtggaagaagacaagaagcatgaacgtcatcctatttttggaaatatagtagatgaagttgcttatcatgagaaatatccaactatctatcatctgcgaaaaaaattggtagattctactgataaagcggatttgcgcttaatctatttggccttagcgcatatgattaagtttcgtggtcattttttgattgagggagatttaaatcctgataatagtgatgtggacaaactatttatccagttggtacaaacctacaatcaattatttgaagaaaaccctattaacgcaagtggagtagatgctaaagcgattctttctgcacgattgagtaaatcaagacgattagaaaatctcattgctcagctccccggtgagaagaaaaatggcttatttgggaatctcattgctttgtcattgggtttgacccctaattttaaatcaaattttgatttggcagaagatgctaaattacagctttcaaaagatacttacgatgatgatttagataatttattggcgcaaattggagatcaatatgctgatttgtttttggcagctaagaatttatcagatgctattttactttcagatatcctaagagtaaatactgaaataactaaggctcccctatcagcttcaatgattaaacgctacgatgaacatcatcaagacttgactcttttaaaagctttagttcgacaacaacttccagaaaagtataaagaaatcttttttgatcaatcaaaaaacggatatgcaggttatattgatgggggagctagccaagaagaattttataaatttatcaaaccaattttagaaaaaatggatggtactgaggaattattggtgaaactaaatcgtgaagatttgctgcgcaagcaacggacctttgacaacggctctattccccatcaaattcacttgggtgagctgcatgctattttgagaagacaagaagacttttatccatttttaaaagacaatcgtgagaagattgaaaaaatcttgacttttcgaattccttattatgttggtccattggcgcgtggcaatagtcgttttgcatggatgactcggaagtctgaagaaacaattaccccatggaattttgaagaagttgtcgataaaggtgcttcagctcaatcatttattgaacgcatgacaaactttgataaaaatcttccaaatgaaaaagtactaccaaaacatagtttgctttatgagtattttacggtttataacgaattgacaaaggtcaaatatgttactgaaggaatgcgaaaaccagcatttctttcaggtgaacagaagaaagccattgttgatttactcttcaaaacaaatcgaaaagtaaccgttaagcaattaaaagaagattatttcaaaaaaatagaatgttttgatagtgttgaaatttcaggagttgaagatagatttaatgcttcattaggtacctaccatgatttgctaaaaattattaaagataaagattttttggataatgaagaaaatgaagatatcttagaggatattgttttaacattgaccttatttgaagatagggagatgattgaggaaagacttaaaacatatgctcacctctttgatgataaggtgatgaaacagcttaaacgtcgccgttatactggttggggacgtttgtctcgaaaattgattaatggtattagggataagcaatctggcaaaacaatattagattttttgaaatcagatggttttgccaatcgcaattttatgcagctgatccatgatgatagtttgacatttaaagaagacattcaaaaagcacaagtgtctggacaaggcgatagtttacatgaacatattgcaaatttagctggtagccctgctattaaaaaaggtattttacagactgtaaaagttgttgatgaattggtcaaagtaatggggcggcataagccagaaaatatcgttattgaaatggcacgtgaaaatcagacaactcaaaagggccagaaaaattcgcgagagcgtatgaaacgaatcgaagaaggtatcaaagaattaggaagtcagattcttaaagagcatcctgttgaaaatactcaattgcaaaatgaaaagctctatctctattatctccaaaatggaagagacatgtatgtggaccaagaattagatattaatcgtttaagtgattatgatgtcgatcacattgttccacaaagtttccttaaagacgattcaatagacaataaggtcttaacgcgttctgataaaaatcgtggtaaatcggataacgttccaagtgaagaagtagtcaaaaagatgaaaaactattggagacaacttctaaacgccaagttaatcactcaacgtaagtttgataatttaacgaaagctgaacgtggaggtttgagtgaacttgataaagctggttttatcaaacgccaattggttgaaactcgccaaatcactaagcatgtggcacaaattttggatagtcgcatgaatactaaatacgatgaaaatgataaacttattcgagaggttaaagtgattaccttaaaatctaaattagtttctgacttccgaaaagatttccaattctataaagtacgtgagattaacaattaccatcatgcccatgatgcgtatctaaatgccgtcgttggaactgctttgattaagaaatatccaaaacttgaatcggagtttgtctatggtgattataaagtttatgatgttcgtaaaatgattgctaagtctgagcaagaaataggcaaagcaaccgcaaaatatttcttttactctaatatcatgaacttcttcaaaacagaaattacacttgcaaatggagagattcgcaaacgccctctaatcgaaactaatggggaaactggagaaattgtctgggataaagggcgagattttgccacagtgcgcaaagtattgtccatgccccaagtcaatattgtcaagaaaacagaagtacagacaggcggattctccaaggagtcaattttaccaaaaagaaattcggacaagcttattgctcgtaaaaaagactgggatccaaaaaaatatggtggttttgatagtccaacggtagcttattcagtcctagtggttgctaaggtggaaaaagggaaatcgaagaagttaaaatccgttaaagagttactagggatcacaattatggaaagaagttcctttgaaaaaaatccgattgactttttagaagctaaaggatataaggaagttaaaaaagacttaatcattaaactacctaaatatagtctttttgagttagaaaacggtcgtaaacggatgctggctagtgccggagaattacaaaaaggaaatgagctggctctgccaagcaaatatgtgaattttttatatttagctagtcattatgaaaagttgaagggtagtccagaagataacgaacaaaaacaattgtttgtggagcagcataagcattatttagatgagattattgagcaaatcagtgaattttctaagcgtgttattttagcagatgccaatttagataaagttcttagtgcatataacaaacatagagacaaaccaatacgtgaacaagcagaaaatattattcatttatttacgttgacgaatcttggagctcccgctgcttttaaatattttgatacaacaattgatcgtaaacgatatacgtctacaaaagaagttttagatgccactcttatccatcaatccatcactggtctttatgaaacacgcattgatttgagtcagctaggaggtgactgaagtatattttagatgaagattatttcttaataactaaaaatatggtataatactcttaataaatgcagtaatacaggggcttttcaagactgaagtctagctgagacaaatagtgcgattacgaaattttttagacaaaaatagtctacgaggttttagagctatgctgttttgaatggtcccaaaactgcagcgcaatagttggcgaagtaatcgcaacatccgcattaaaatctagcgagggctttactaagctccgcaaaaaaccccgcccctgacagggcggggttttttcgcgcccgatccttggagcccttgccctcccgcacgatgatcgtgccgtgatcgaaatccagatccttgacccgcagttgcaaaccctcactgatccgcatgcttatgacaacttgacggctacatcattcactttttcttcacaaccggcacggaactcgctcgggctggccccggtgcattttttaaatacccgcgagaaatagagttgatcgtcaaaaccaacattgcgaccgacggtggcgataggcatccgggtggtgctcaaaagcagcttcgcctggctgatacgttggtcctcgcgccagcttaagacgctaatccctaactgctggcggaaaagatgtgacagacgcgacggcgacaagcaaacatgctgtgcgacgctggcgatatcaaaattgctgtctgccaggtgatcgctgatgtactgacaagcctcgcgtacccgattatccatcggtggatggagcgactcgttaatcgcttccatgcgccgcagtaacaattgctcaagcagatttatcgccagcagctccgaatagcgcccttccccttgcccggcgttaatgatttgcccaaacaggtcgctgaaatgcggctggtgcgcttcatccgggcgaaagaaccccgtattggcaaatattgacggccagttaagccattcatgccagtaggcgcgcggacgaaagtaaacccactggtgataccattcgcgagcctccggatgacgaccgtagtgatgaatctctcctggcgggaacagcaaaatatcacccggtcggcaaacaaattctcgtccctgatttttcaccaccccctgaccgcgaatggtgagattgagaatataacctttcattcccagcggtcggtcgataaaaaaatcgagataaccgttggcctcaatcggcgttaaacccgccaccagatgggcattaaacgagtatcccggcagcaggggatcattttgcgcttcagccatacttttcatactcccgccattcagagaagaaaccaattgtccatattgcatcagacattgccgtcactgcgtcttttactggctcttctcgctaaccaaaccggtaaccccgcttattaaaagcattctgtaacaaagcgggaccaaagccatgacaaaaacgcgtaacaaaagtgtctataatcacggcagaaaagtccacattgattatttgcacggcgtcacactttgctatgccatagcatttttatccataagattagcggatcctacctgacgctttttatcgcaactctctactgtttctccatgtaggtcgttcgctccaagcgttttagagctagaaatagcaagttaaaataaggctagtccgttatcaacttgaaaaagtggcaccagaccccgttgatgataccgctgccttactgggtgcattagccagtctgaatgacctcgagttttagagctatgctgttttgaatggtcccaaaacttcagcacactgagacttgttgagttccatgttttagagctatgctgttttgaatggactccattcaacattgccgatgataacttgagaaagagggttaataccagcagtcggataccttcctattctttctgttaaagcgttttcatgttataataggcaaaagaagagtagtgtgatcgtccattccgacgtcgagccgttccatacagaagctgggcgaacaaacgatgctcgccttccagaaaaccgaggatgcgaaccacttcatccggggtcagcaccaccggcaagcgccgcgacggccgaggtcttccgatctcctgaagccagggcagatccgtgcacagcaccttgccgtagaagaacagcaaggccgccaatgcctgacgatgcgtggagaccgaaaccttgcgctcgttcgccagccaggacagaaatgcctcgacttcgctgctgcccaaggttgccgggtgacgcacaccgtggaaacggatgaaggcacgaacccagtggacataagcctgttcggttcgtaagctgtaatgcaagtagcgtatgcgctcacgcaactggtccagaaccttgaccgaacgcagcggtggtaacggcgcagtggcggttttcatggcttgttatgactgtttttttggggtacagtctatgcctcgggcatccaagcagcaagcgcgttacgccgtgggtcgatgtttgatgttatggagcagcaacgatgttacgcagcagggcagtcgccctaaaacaaagttaaacatcatgagggaagcggtgatcgccgaagtatcgactcaactatcagaggtagttggcgtcatcgagcgccatctcgaaccgacgttgctggccgtacatttgtacggctccgcagtggatggcggcctgaagccacacagtgatattgatttgctggttacggtgaccgtaaggcttgatgaaacaacgcggcgagctttgatcaacgaccttttggaaacttcggcttcccctggagagagcgagattctccgcgctgtagaagtcaccattgttgtgcacgacgacatcattccgtggcgttatccagctaagcgcgaactgcaatttggagaatggcagcgcaatgacattcttgcaggtatcttcgagccagccacgatcgacattgatctggctatcttgctgacaaaagcaagagaacatagcgttgccttggtaggtccagcggcggaggaactctttgatccggttcctgaacaggatctatttgaggcgctaaatgaaaccttaacgctatggaactcgccgcccgactgggctggcgatgagcgaaatgtagtgcttacgttgtcccgcatttggtacagcgcagtaaccggcaaaatcgcgccgaaggatgtcgctgcctactgggcaatggagcgcctgccggcccagtatcagcccgtcatacttgaagctagacaggcttatcttggacaagaagaagatcgcttggcctcgcgcgcagatcagttggaagaatttgtccactacgtgaaaggcgagatcaccaaggtagtcggcaaataatgtctaacaattcgttcaagccgacgccgcttcgcggcgcggcttaactcaagcgttagatgcactaagcacataattgctcacagccaaactatcaggtcaagtctgcttttattatttttaagcgtgcataataagccctacacaaattgggagatatatcatgaaaggctggctttttcttgttatcgcaatagttggcgaagtaatcgcaacatccgcattaaaatctagcgagggctttactaagctcctgcagagatctgaattccctagagagacgaaagtgattgcgcctacccggatattatcgtgaggatgcgtcatcgccattgctccccaaatacaaaaccaatttcagccagtgcctcgtccattttttcgatgaactccggcacgatctcgtcaaaactcgccatgtacttttcatcccgctcaatcacgacataatgcaggccttcacgcttcatacgcgggtcatagttggcaaagtaccaggcattttttcgcgtcacccacatgctgtactgcacctgggccatgtaagctgactttatggcctcgaaaccaccgagccggaacttcatgaaatcccgggaggtaaacgggcatttcagttcaaggccgttgccgtcactgcataaaccatcgggagagcaggcggtacgcatactttcgtcgcgatagatgatcggggattcagtaacattcacgccggaagtgaattcaaacagggttctggcgtcgttctcgtactgttttccccaggccagtgctttagcgttaacttccggagccacaccggtgcaaacctcagcaagcagggtgtggaagtaggacattttcatgtcaggccacttctttccggagcggggttttgctatcacgttgtgaacttctgaagcggtgatgacgccgagccgtaatttgtgccacgcatcttccccctgttcgacagctctcacatcgatcccggtacgctgcaggataatgtccggtgtcatgctgccaccttctgctctgcggctttctgtttcaggaatccaagagcttttactgcttcggcctgtgtcagttctgacgatgcacgaatgtcgcggcgaaatatctgggaacagagcggcaataagtcgtcatcccatgttttatccagggcgatcagcagagtgttaatctcctgcatggtttcatcgttaaccggagtgatgtcgcgttccggctgacgttctgcagtgtatgcagtattttcgacaatgcgctcggcttcatccttgtcatagataccagcaaatccgaaggccagacgggcacactgaatcatggctttatgacgtaacatccgtttgggatgcgactgccacggccccgtgatttctctgccttcgcgagttttgaatggttcgcggcggcattcatccatccattcggtaacgcagatcggatgattacggtccttgcggtaaatccggcatgtacaggattcattgtcctgctcaaagtccatgccatcaaactgctggttttcattgatgatgcgggaccagccatcaacgcccaccaccggaacgatgccattctgcttatcaggaaaggcgtaaatttctttcgtccacggattaaggccgtactggttggcaacgatcagtaatgcgatgaactgcgcatcgctggcatcacctttaaatgccgtctggcgaagagtggtgatcagttcctgtgggtcgacagaatccatgccgacacgttcagccagcttcccagccagcgttgcgagtgcagtactcattcgttttatacctctgaatcaatatcaacctggtggtgagcaatggtttcaaccatgtaccggatgtgttctgccatgcgctcctgaaactcaacatcgtcatcaaacgcacgggtaatggattttttgctggccccgtggcgttgcaaatgatcgatgcatagcgattcaaacaggtgctggggcaggcctttttccatgtcgtctgccagttctgcctctttctcttcacgggcgagctgctggtagtgacgcgcccagctctgagcctcaagacgatcctgaatgtaataagcgttcatggctgaactcctgaaatagctgtgaaaatatcgcccgcgaaatgccgggctgattaggaaaacaggaaagggggttagtgaatgcttttgcttgatctcagtttcagtattaatatccattttttataagcgtcgactgtttcctgtgtgaaattgttatccgctcacaattccacacattatacgagccggaagcataaagtgtaaagcctggggtgcctaatgagtgagaattcggatctcgacgggatgttgattctgtcatggcatatccttacaacttaaaaaagcaaaagggccgcagatgcgacccttgtgtatcaaacaagacgattaaaaatcttcgttagtttctgctacgccttcgctatcatctacagagaaatccggcgttgagttcgggttgctcagcagcaactcacgtactttcttctcgatctctttcgcggtttccgggttatctttcagccaggcagtcgcattcgctttaccctgaccgatcttctcacctttgtagctgtaccacgcgcctgctttctcgatcagcttctcttttacgcccaggtcaaccagttcgccgtagaagttgataccttcgccgtagaggatctggaattcagcctgtttaaacggcgcagcgattttgttcttcaccactttcacgcgggtttcgctacccaccacgttttcgccctctttcaccgcgccgatacgacggatgtcgagacgaacagaggcgtagaatttcagcgcgttaccaccggtagtggtttccgggttaccgaacatcacaccaattttcatacggatctggttgatgaagatcagcagcgtgttggactgcttcaggttacccgccagcttacgcatcgcctggctcatcatacgtgccgcaaggcccatgtgagagtcgccgatttcgccttcgatttccgctttcggcgtcagtgccgccacggagtcaacgacgataacgtctactgcgccagaacgcgccagggcgtcacagatttccagtgcctgctcgccggtgtccggctgggagcacagcaggttgtcgatatcgacgcccagtttacgtgcgtagattgggtccagcgcgtgttcagcatcgataaacgcacaggttttaccttcacgctgcgctgcggcgatcacctgcagcgtcagcgtggttttaccggaagattccggtccgtagatttcgacgatacggcccatcggcagaccacctgccccaagcgcgatatccagtgaaagcgaaccggtagagatggtttccacatccatggaacggtcttcacccaggcgcatgatggagcctttaccaaattgtttctcaatctggcccagtgctgccgccaacgctttctgtttgttttcgtcgatagccatttttactcctgtcatgccgggtaataccggatagtcaatatgttctgttgaagcaattatactgtatgctcatacagtatcaagtgttttgtagaaattgttgccacaaggtctgcaatgcatacgcagtagcctgacgacgcaccgcatcacggtcgccgctgaagcatcccgccgggtaatgccttcaccgcgggcagtggcaaaagcaaaccagacggtgccgacaggcttctctagatccgcctacctttcacgagttgcgcagtttgtctgcaagactctatgagaagcagataagcgataagtttgctcaacatcttctcgggcataagtcggacaccatggcatcacagtatcgtgatgacagaggcagggagtgggacaaaattgaaatcaaataatgattttattttgactgatagtgacctgttcgttgcaacaaattgataagcaatgccaagcttggcactggctgatcagctagctcactgcccgctttccagtcgggaaacctgtcgtgccagctgcattaatgaatcggccaacgcgcggggagaggcggtttgcgtattgggcgccagggtggtttttcttttcaccagtgagacgggcaacagctgattgcccttcaccgcctggccctgagagagttgcagcaagcggtccacgctggtttgccccagcaggcgaaaatcctgtttgatggtggttaacggcgggatataacatgagctgtcttcggtatcgtcgtatcccactaccgagatatccgcaccaacgcgcagcccggactcggtaatggcgcgcattgcgcccagcgccatctgatcgttggcaaccagcatcgcagtgggaacgatgccctcattcagcatttgcatggtttgttgaaaaccggacatggcactccagtcgccttcccgttccgctatcggctgaatttgattgcgagtgagatatttatgccagccagccagacgcagacgcgccgagacagaacttaatgggcccgctaacagcgcgatttgctggtgacccaatgcgaccagatgctccacgcccagtcgcgtaccgtcttcatgggagaaaataatactgttgatgggtgtctggtcagagacatcaagaaataacgccggaacattagtgcaggcagcttccacagcaatggcatcctggtcatccagcggatagttaatgatcagcccactgacgcgttgcgcgagaagattgtgcaccgccgctttacaggcttcgacgccgcttcgttctaccatcgacaccaccacgctggcacccagttgatcggcgcgagatttaatcgccgcgacaatttgcgacggcgcgtgcagggccagactggaggtggcaacgccaatcagcaacgactgtttgcccgccagttgttgtgccacgcggttgggaatgtaattcagctccgccatcgccgcttccactttttcccgcgttttcgcagaaacgtggctggcctggttcaccacgcgggaaacggtctgataagagacaccggcatactctgcgacatcgtataacgttactggtttcacattcaccaccctgaattgactctcttccgggcgctatcatgccataccgcgaaaggttttgcaccattcgatgctagcccatgggtatggacagttttccctttgatatgtaacggtgaacagttgttctacttttgtttgttagtcttgatgcttcactgatagatacaagagccataagaacctcagatccttccgtatttagccagtatgttctctagtgtggttcgttgtttttgcgtgagccatgagaacgaaccattgagatcatacttactttgcatgtcactcaaaaattttgcctcaaaactggtgagctgaatttttgcagttaaagcatcgtgtagtgtttttcttagtccgttacgtaggtaggaatctgatgtaatggttgttggtattttgtcaccattcatttttatctggttgttctcaagttcggttacgagatccatttgtctatctagttcaacttggaaaatcaacgtatcagtcgggcggcctcgcttatcaaccaccaatttcatattgctgtaagtgtttaaatctttacttattggtttcaaaacccattggttaagccttttaaactcatggtagttattttcaagcattaacatgaacttaaattcatcaaggctaatctctatatttgccttgtgagttttcttttgtgttagttcttttaataaccactcataaatcctcatagagtatttgttttcaaaagacttaacatgttccagattatattttatgaatttttttaactggaaaagataaggcaatatctcttcactaaaaactaattctaatttttcgcttgagaacttggcatagtttgtccactggaaaatctcaaagcctttaaccaaaggattcctgatttccacagttctcgtcatcagctctctggttgctttagctaatacaccataagcattttccctactgatgttcatcatctgagcgtattggttataagtgaacgataccgtccgttctttccttgtagggttttcaatcgtggggttgagtagtgccacacagcataaaattagcttggtttcatgctccgttaagtcatagcgactaatcgctagttcatttgctttgaaaacaactaattcagacatacatctcaattggtctaggtgattttaatcactataccaattgagatgggctagtcaatgataattactagtccttttcctttgagttgtgggtatctgtaaattctgctagacctttgctggaaaacttgtaaattctgctagaccctctgtaaattccgctagacctttgtgtgttttttttgtttatattcaagtggttataatttatagaataaagaaagaataaaaaaagataaaaagaatagatcccagccctgtgtataactcactactttagtcagttccgcagtattacaaaaggatgtcgcaaacgctgtttgctcctctacaaaacagaccttaaaaccctaaaggcttaagtagcaccctcgcaagctcggttgcggccgcaatcgggcaaatcgctgaatattccttttgtctccgaccatcaggcacctgagtcgctgtctttttcgtgacattcagttcgctgcgctcacggctctggcagtgaatgggggtaaatggcactacaggcgccttttatggattcatgcaaggaaactacccataatacaagaaaagcccgtcacgggcttctcagggcgttttatggcgggtctgctatgtggtgctatctgactttttgctgttcagcagttcctgccctctgattttccagtctgaccacttcggattatcccgtgacaggtcattcagactggctaatgcacccagtaaggcagcggtatcatcaacggggtctgacgctcagtggaacgaaaactcacgttaagggattttggtcatgagattatcaaaaaggatcttcacctagatccttttaaattaaaaatgaagttttaaatcaatctaaagtatatatgagtaaacttggtctgacagttaccaatgcttaatcagtgaggcacctatctcagcgatctgtctatttcgttcatccatagttgcctgactccccgtcgtgtagataactacgatacgggagggcttaccatctggccccagtgctgcaatgataccgcgagacccacgctcaccggctccagatttatcagcaataaaccagccagccg

SEQ ID NO: 137 - DNA, 3240 bp, synthetic construct
  source 1..3240: mol_type = other DNA
ccacctgacgtctaagaaaccattattatcatgacattaacctataaaaataggcgtatcacgaggcagaatttcagataaaaaaaatccttagctttcgctaaggatgatttctggaattcgcggccgcatctagagtctcgagttgacagctagctcagtcctaggtataatgctagcctcgaggaaagaggagaaaggtctcaatgcgtaaaggcgaagagctgttcactggtgtcgtccctattctggtggaactggatggtgatgtcaacggtcataagttttccgtgcgtggcgagggtgaaggtgacgcaactaatggtaaactgacgctgaagttcatctgtactactggtaaactgccggtaccttggccgactctggtaacgacgctgacttatggtgttcagtgctttgctcgttatccggaccatatgaagcagcatgacttcttcaagtccgccatgccggaaggctatgtgcaggaacgcacgatttcctttaaggatgacggcacgtacaaaacgcgtgcggaagtgaaatttgaaggcgataccctggtaaaccgcattgagctgaaaggcattgactttaaagaagacggcaatatcctgggccataagctggaatacaattttaacagccacaatgtttacatcaccgccgataaacaaaaaaatggcattaaagcgaattttaaaattcgccacaacgtggaggatggcagcgtgcagctggctgatcactaccagcaaaacactccaatcggtgatggtcctgttctgctgccagacaatcactatctgagcacgcaaagcgttctgtctaaagatccgaacgagaaacgcgatcatatggttctgctggagttcgtaaccgcagcgggcatcgcgcatggtatggatgaactgtacagatgataacgctgatagtgctagtgtagatcgctactagagccaggcatcaaataaaacgaaaggctcagtcgaaagactgggcctttcgttttatctgttgtttgtcggtgaacgctctctactagagtcacactggctcaccttcgggtgggcctttctgcgtttatatactagaagcggccgctgcaggaattcaaaaaaagcaccgactcggtgccactttttcaagttgataacggactagccttattttaacttgctatttctagctctaaaacggagacgagcgtctccactagtattatacctaggactgagctagctgtcaaggatccagcatatgcggtgtgaaataccgcacagatgcgtaaggagaaaataccgcatcaggcgctcttccgcttcctcgctcactgactcgctgcgctcggtcgttcggctgcggcgagcggtatcagctcactcaaaggcggtaatacggttatccacagaatcaggggataacgcaggaaagaacatgtgagcaaaaggccagcaaaaggccaggaaccgtaaaaaggccgcgttgctggcgtttttccataggctccgcccccctgacgagcatcacaaaaatcgacgctcaagtcagaggtggcgaaacccgacaggactataaagataccaggcgtttccccctggaagctccctcgtgcgctctcctgttccgaccctgccgcttaccggatacctgtccgcctttctcccttcgggaagcgtggcgctttctcatagctcacgctgtaggtatctcagttcggtgtaggtcgttcgctccaagctgggctgtgtgcacgaaccccccgttcagcccgaccgctgcgccttatccggtaactatcgtcttgagtccaacccggtaagacacgacttatcgccactggcagcagccactggtaacaggattagcagagcgaggtatgtaggcggtgctacagagttcttgaagtggtggcctaactacggctacactagaaggacagtatttggtatctgcgctctgctgaagccagttaccttcggaaaaagagttggtagctcttgatccggcaaacaaaccaccgctggtagcggtggtttttttgtttgcaagcagcagattacgcgcagaaaaaaaggatctcaagaagatcctttgatcttttctacggggtctgacgctcagtggaacgaaaactcacgttaagggattttggtcatgagattatcaaaaaggatcttcacctagatccttttaaattaaaaatgaagttttaaatcaatctaaagtatatatgagtaaacttggtctgacagttaccaatgcttaatcagtgaggcacctatctcagcgatctgtctatttcgttcatccatagttgcctgactccccgtcgtgtagataactacgatacgggagggcttaccatctggccccagtgctgcaatgataccgcgtgacccacgctcaccggctccagatttatcagcaataaaccagccagccggaagggccgagcgcagaagtggtcctgcaactttatccgcctccatccagtctattaattgttgccgggaagctagagtaagtagttcgccagttaatagtttgcgcaacgttgttgccattgctacaggcatcgtggtgtcacgctcgtcgtttggtatggcttcattcagctccggttcccaacgatcaaggcgagttacatgatcccccatgttgtgcaaaaaagcggttagctccttcggtcctccgatcgttgtcagaagtaagttggccgcagtgttatcactcatggttatggcagcactgcataattctcttactgtcatgccatccgtaagatgcttttctgtgactggtgagtactcaaccaagtcattctgagaatagtgtatgcggcgaccgagttgctcttgcccggcgtcaatacgggataataccgcgccacatagcagaactttaaaagtgctcatcattggaaaacgttcttcggggcgaaaactctcaaggatcttaccgctgttgagatccagttcgatgtaacccactcgtgcacccaactgatcttcagcatcttttactttcaccagcgtttctgggtgagcaaaaacaggaaggcaaaatgccgcaaaaaagggaataagggcgacacggaaatgttgaatactcatactcttcctttttcaatattattgaagcatttatcagggttattgtctcatgagcggatacatatttgaatgtatttagaaaaataaacaaataggggttccgcgcacatttccccgaaaagtg

SEQ ID NO: 138 - DNA, 6558 bp, synthetic construct
  source 1..6558: mol_type = other DNA
gcatgctcaaggcctgacaaaccctgtcgtttttcgccaactcctgcgaggtaacctcgaacatgcgctgtaagttggcgtagctgtcctgccacgcttgctgctgttgttcgtagtgcctctgtaagctctctaatgcgctcagaagctgctgctccatttcggtcatgaatctcttcaccctgatagataaaaccgcccagaatcgattctgtggcgtctgatgaggttatttggcgctgtacttgatgacctgacgatgttgagcgttcttgtactcgtcgatcttcttcgccccctgcggaaggatcaggtaatacacgctcttgttcttggaatcgtgaattatcgatacgccggctccggtctggctctttaagtcctgcaggatctggctctgctcgctgatttcgttctggcgttcgaccacgatagtcccgagataccaagctactccaatcaatatcgcaaacaggatcccacttaatgccaggctgtacagccatgtcattccgactaagcggtgtatctgttttagctggctgtcgttctcttcttggatagcggtctgtatgttccctgagcttaatttcaaggcctcggtgatacgtttctcgtgcttctcgaatgcgttcgcgacgctcgttgcggtagtcttggcttgctgcttcgatttgctctcgaactcccgcgctaaatttaaaatctcgctcatacagcactccttttaagcgaatattcgggccacctgccggatcagcaatactgatactggatttggtttcccgtacgaccgacaatccggcatcggtaaggtgggaaatcacccctttacgatccgtaatttctccctgctcaatcaagctgattagccctttggtaatggcttccgctgcctgctgtttgttgcgaggaaggtcattagagggggttaatgctcggcgattagcagggtcattcgggtcgcgtaacccaagccggtcattggtgagggtttgccatgcgttaacacgaggccggtcagcccgatcaaagtaaggttgtagccgttttccgctctgcaattcgatgttcgggataacaaaattcaattcaagacgccctttgtcctgatgttgaacccagaggcaggcatactggtctttatctagaccggtcatcaatgtctgctcccattcatccatcaatcgctgcttttcgccttcgggtaaatcactctcctgaaaagagagcacgccagaggtataagttcgggcaaattcgcagccatcaatcagctctttgacgtgctcagggttaccccgtaacaccgtcgcttgttcgcgctgacgatcagggcccagaaggtaatcgacaggaccactcccgccaccggcaccacgaccatgaatcttaacgatcacgatgttgctccagcagttcggcaagatgttggtcaatgctattgagcaccgctaacaacgacacccgttcttgcggcggtaagccatgctgattcaagtaacgggctatttgattgaggttattaccgatcccgctgacctgacgtaacaaggtcgggtctacggtaggtagcggacgacgccgagctgtacgcgattcgcctaagccaacggctcgtaaccactcggccaaatgcttacggtcacagcgttcaagtagccgctgatgctccgcttcggtgagtctgattttgatctctttggtgcgcttttccatgagaatccgctgagaaagtttcgcacccaaagtgcgaattttcgcagtggatgcaaggggtttcggggggcggcgagccccctgaaacagtcacagacggcacctcgaagaggggacgctgtgtgtactggcttagtacagcatctatcgtacatcgaggtcgcatcacgcacaaacaaaaagccccgcaaaagcagggctgttatctgatataggttgttttgtctcacacggcagcggaagaggaatccgaagtggtactggtagtagtattggatgctgctgacgatattttccgctttgacccaaggcttaaataatcaatgcctgtaatcaacgatctcaatacgccttcggataccatagcgataaacgtatcttgctggttatggcttgcgatgcaaatcgtagcatcaccttttttatactttaaaacacctgctaaatatccattttcatctagaacactcttaagatgttcatttgttattgtttgtagcgtttgctttgtttcgcttcgagcatacgccttagctagcttccgagaaaaagcatccgcatcatgactatctttatttactcgctcaataaatttgcttaagtcaacaaatcccttaaaacgagtggacatattgttaacaaaatcagtggcagcattttttatccatgctttatagccaaaaaaacgctcgaaaacattttggtcgtagataaataccgtatcgccagcaaaaacaagagatgccttaccatcaatagaaatcatatcttgatctactcgagatagttcttttttgctaaacccataaaaattatttttctttcttgataagttttgaactggatattgcttcttgtatatggttatacaattgtcgtcattattcttactcaaaacgaaaatgattgagtcaacttttgatattagatccacactgtcaaaatcaacaattgggatattttcattgccatcaccaccaaacccagcatcaaacacaatgccagtcagaaacttcatttgctcattatcatactgctcagcatcatttaaaaatgaaatggtgttggtgcggtcacttagtgtattaacatctgatactatcacaacccgattttctaaatcagatatagttttctttatcacattatcaataatggactgttttagctcactgtcatttttaaggatggcaattttatagctaaaagagtccttagcacccgctttacctttatttttaaagttaaagtaagtgtgcaatgtaacatcgttaatatcacaatcaaaatgcttatacagttctaaaagctcttgtgctttttcttcattatgctccaaagcatcaagatctggaattcgcggccgcatctagagtctcgagttgacagctagctcagtcctaggtataatgctagcctcgaggaaagaggagaaaggtctcaatgagccatattcaacgggaaacgtcttgctctaggccgcgattaaattccaacatggatgctgatttatatgggtataaatgggctcgcgataatgtcgggcaatcaggtgcgacaatctatcgattgtatgggaagcccgatgcgccagagttgtttctgaaacatggcaaaggtagcgttgccaatgatgttacagatgagatggtcagactaaactggctgacggaatttatgcctcttccgaccatcaagcattttatccgtactcctgatgatgcatggttactcaccactgcgatccccgggaaaacagcattccaggtattagaagaatatcctgattcaggtgaaaatattgttgatgcgctggcagtgttcctgcgccggttgcattcgattcctgtttgtaattgtccttttaacagcgatcgcgtatttcgtctcgctcaggcgcaatcacgaatgaataacggtttggttgatgcgagtgattttgatgacgagcgtaatggctggcctgttgaacaagtctggaaagaaatgcataaacttttgccattctcaccggattcagtcgtcactcatggtgatttctcacttgataaccttatttttgacgaggggaaattaataggttgtattgatgttggacgagtcggaatcgcagaccgataccaggatcttgccatcctatggaactgcctcggtgagttttctccttcattacagaaacggctttttcaaaaatatggtattgataatcctgatatgaataaattgcagtttcatttgatgctcgatgagtttttctaataacgctgatagtgctagtgtagatcgctactagagccaggcatcaaataaaacgaaaggctcagtcgaaagactgggcctttcgttttatctgttgtttgtcggtgaacgctctctactagagtcacactagatctaaggcatcgtcactcatcatcattcctctatgatttttttcgcgaacgttaaataatcatcatgatttataactctgataaaatcattttcttttattaaatctttagataaaactatcaactcaccgtcttgcgttttttcccttccattagctaccacactgtaagtaatcttataggcagaaacattaaataatgacaatgttgggttgcagtgaattctttttgttttgatgtgcaaaaaaccgacgataatcaaaacaaacaaaaaattaactatatttgatggtttgcttaaatcagtaaagaccaacggcattatgtacgttgataaaaaagaaagatactcaccggattcttttttacatgaaacgacctttaactttcttgacaccgcaccggagtctaagtttttcaaaacccatcgataccaaatgtatgtataagaacaagttaaaatcaaagccccgcagatcactgacctcaatacagaaaatgttaatctgctatttgaatagtcgagtacgcattgaaattttccatccgcgccagaacacgaagacatggccttatctaaaacagaccatacgttatcaataccagaaaaatatattgttatcggtataaataaaaacaacattgataagagatacattctaattttcatttttgtaaaatttcctgtaccacgttgatctacttattcctaaagaaatccattctccatctctaactttcggccttccaccaccagagcttttttttccacgttgacgctgaatttcagaagtatgtgtttgtttaacatactcttcaaagccaagctctgtaaggttcttacttgtccacttagccacacttttagcaattcccatgacttcgttctcgtctaaaggtgcggagaactgcaggttgtaggctttagcgcgttcaatgcaggcttgtagccattggtcatactgcggccagccttggcggatagcgcggtaagcccacttgcgggttttatcgaagagggtgcagttacggcctaaaccgtagtccggcaggatttcgcggtcattggctgcgccaaggtcgaggtaatcggctaaccagtcaagggtatagagctctggctgccagacggtgatctgccagtgcaggtggttcggattcttgcaaattagccctgaataccccgcatctgcgcccaattttttacgcagcgcattctcgatggcggcggcgtatttaaggggggcagctcgaccatccggcgcggtacgtaccgccgtatgcaaggcatacaacaggtgagcatgtccgttctcggggtttttgatggtgagtgtgggcgcaggtgcccccagatcggcccaatcaatcgcggctccggctctgtccacgtcaaagcaaagccagtacatggcgtgaggctgattaaactggatgtattttgcgaggagagcacgctctttaccggcaatgcgaacaccaaactgtaaatcatcggagaagtacggcttgtggggtaaccggtcgttaaaaagcgttaaagcctgattatccaaggctcccagccttatggcggggctgttgttttgcacgctgcatgtgctaatatcctttctaggtttcgacctagccctgaatgtcatgtccgctcgccaaagtagagcatgatttcggggctttgttttttctgccactaagttacacctcaacaacggtttttgtcatccccgacaatccgttattcctgcttgttctcgcacggctttacgctcatactacttcttgtagatacacttgtcactacatcaagaggtgagatgatggccacgattaatattcggatcgatgacgagctgaaaagccgctcttatgccgcactggaaaagctgggcgtaacgccgtccgaggttctgcgccaaacactggaatatgtggcccaaagcggacgtttgccgttccagcaggttttgctgaccgaggatgatgccgatttgatggctatcgttcgggatcgtctggaaaacccacaggcgggcgtaaaggtgtcactggatgagctataaccttgaatttgatccccgagccctgaaggaatggcgcaagctcggggatgatgtccgtctgcagttcaagaaaaaactcgagcaggttctacaacacccgcggatcgataaaaatcgcctgcgagagctgcatgactgctacaaaatcaagctccgtgcatccggttatcgcttggtctatcaggttcgcgatcaaaccattacggtattcgtggtggcggtcggtaagcgcgagcgttctgccgcttacgatgcggccgataaacgcttataaactcatgccgtgaccgcgagaataccgctgttcgtgccgcttggctaattgctcaagcggcgcactgttctgtttaagctctcgacttgctgcgccaagccggtgactt

SEQ ID NO: 139 - DNA, 1231 bp, synthetic construct
  source 1..1231: mol_type = other DNA
tctagagcttgtcgacgtctcgagtttacagctagctcagtcctaggtattatgctagcctcgaggaaagaggagaaagaagcttaagaaaaagatcattagcgcgatcctgatgagcaccgtgattctgagcgcggcggcgccgctgagcggtgtttatgcgattgttaacagcaagcgtagcgagctggataagaaaatcagcattgcggcgaaagagatcaagagcgcgaacgcggcggaaattaccccgagccgtagcagcaacgaggaactggagaaagaactgaaccgttacgcgaaggcggttggtagcctggaaaccgcgtataaaccgtttctggcgagcagcgcgctggtgccgaccaccccgaccgcgttccaaaacgagctgaaaacctttcgtgacagcctgatcagcagctgcaagaaaaagaacatcctgattaccgataccagcagctggctgggcttccaggtttacagcacccaagcgccgagcgtgcaggcggcgagcaccctgggttttgagctgaaagcgattaacagcctggttaacaagctggcggaatgcggcctgagcaaattcatcaaggtgtatcgtccgcagctgccgattgaaaccccggcgaacaacccggaggaaagcgacgaagcggatcaggcgccgtggaccccgatgccgctggagatcgcgttccagggtgaccgtgaaagcgttctgaaagcgatgaacgcgattaccggcatgcaagattacctgtttaccgtgaacagcatccgtattcgtaacgaacgtatgatgccgccgccaatcgcgaacccggctgcggcgaagccggctgcggcgcagccggcgaccggtgcggcgagcctgaccccggcggacgaggctgcggcgccggctgcgccggcgatccagcaagttattaaaccggctatgggcaaggaacaggtgttcgttcaagtgagcctgaacctggtgcactttaaccagccgaaagcgcaagagccgagcgaagatcatcatcaccaccaccactaacgagctcgatagtgctagtgtagatcgctactagagccaggcatcaaataaaacgaaaggctcagtcgaaagactgggcctttcgttttatctgttgtttgtcggtgaacgctctctactagagtcacactggctcaccttcgggtgggcctttctgcgtttatatactagaagcggccgctgcag

SEQ ID NO: 140 - DNA, 1231 bp, synthetic construct
  source 1..1231: mol_type = other DNA
tctagagcttgtcgacgtctcgagtttacggctagctcagtcctaggtacaatgctagcctcgaggaaagaggagaaagaagcttaagaaaaagatcattagcgcgatcctgatgagcaccgtgattctgagcgcggcggcgccgctgagcggtgtttatgcgattgttaacagcaagcgtagcgagctggataagaaaatcagcattgcggcgaaagagatcaagagcgcgaacgcggcggaaattaccccgagccgtagcagcaacgaggaactggagaaagaactgaaccgttacgcgaaggcggttggtagcctggaaaccgcgtataaaccgtttctggcgagcagcgcgctggtgccgaccaccccgaccgcgttccaaaacgagctgaaaacctttcgtgacagcctgatcagcagctgcaagaaaaagaacatcctgattaccgataccagcagctggctgggcttccaggtttacagcacccaagcgccgagcgtgcaggcggcgagcaccctgggttttgagctgaaagcgattaacagcctggttaacaagctggcggaatgcggcctgagcaaattcatcaaggtgtatcgtccgcagctgccgattgaaaccccggcgaacaacccggaggaaagcgacgaagcggatcaggcgccgtggaccccgatgccgctggagatcgcgttccagggtgaccgtgaaagcgttctgaaagcgatgaacgcgattaccggcatgcaagattacctgtttaccgtgaacagcatccgtattcgtaacgaacgtatgatgccgccgccaatcgcgaacccggctgcggcgaagccggctgcggcgcagccggcgaccggtgcggcgagcctgaccccggcggacgaggctgcggcgccggctgcgccggcgatccagcaagttattaaaccggctatgggcaaggaacaggtgttcgttcaagtgagcctgaacctggtgcactttaaccagccgaaagcgcaagagccgagcgaagatcatcatcaccaccaccactaacgagctcgatagtgctagtgtagatcgctactagagccaggcatcaaataaaacgaaaggctcagtcgaaagactgggcctttcgttttatctgttgtttgtcggtgaacgctctctactagagtcacactggctcaccttcgggtgggcctttctgcgtttatatactagaagcggccgctgcag

SEQ ID NO: 141 - DNA, 1245 bp, synthetic construct
  source 1..1245: mol_type = other DNA
tctagagcttgtcgacgtctcgagtttacagctagctcagtcctaggtattatgctagcctcgaggaaagaggagaaagaagcttatgaagaaaaagatcattagcgcgatcctgatgagcaccgtgattctgagcgcggcggcgccgctgagcggtgtttatgcgggtagcagccatcatcaccaccaccacgacgacgacgacaaaattgttaacagcaagcgtagcgagctggataagaaaatcagcattgcggcgaaagagatcaagagcgcgaacgcggcggaaattaccccgagccgtagcagcaacgaggaactggagaaagaactgaaccgttacgcgaaggcggttggtagcctggaaaccgcgtataaaccgtttctggcgagcagcgcgctggtgccgaccaccccgaccgcgttccaaaacgagctgaaaacctttcgtgacagcctgatcagcagctgcaagaaaaagaacatcctgattaccgataccagcagctggctgggcttccaggtttacagcacccaagcgccgagcgtgcaggcggcgagcaccctgggttttgagctgaaagcgattaacagcctggttaacaagctggcggaatgcggcctgagcaaattcatcaaggtgtatcgtccgcagctgccgattgaaaccccggcgaacaacccggaggaaagcgacgaagcggatcaggcgccgtggaccccgatgccgctggagatcgcgttccagggtgaccgtgaaagcgttctgaaagcgatgaacgcgattaccggcatgcaagattacctgtttaccgtgaacagcatccgtattcgtaacgaacgtatgatgccgccgccaatcgcgaacccggctgcggcgaagccggctgcggcgcagccggcgaccggtgcggcgagcctgaccccggcggacgaggctgcggcgccggctgcgccggcgatccagcaagttattaaaccgtatatgggcaaggaacaggtgttcgttcaagtgagcctgaacctggtgcactttaaccagccgaaagcgcaagagccgagcgaagattgacgagctcgatagtgctagtgtagatcgctactagagccaggcatcaaataaaacgaaagactgggcctttcgttttatctgttgtttgtcggtgaacgctctctactagagtcacactggctcaccttcgggtgggcctttctgcgtttatatactagaagcggccgctgcag

SEQ ID NO: 142 - DNA, 1258 bp, synthetic construct
  source 1..1258: mol_type = other DNA
tctagagcttgtcgacgtctcgagtttacggctagctcagtcctaggtacaatgctagcctcgaggaaagaggagaaagaagcttatgaagaaaaagatcattagcgcgatcctgatgagcaccgtgattctgagcgcggcggcgccgctgagcggtgtttatgcgggtagcagccatcatcaccaccaccacgacgacgacgacaaaattgttaacagcaagcgtagcgagctggataagaaaatcagcattgcggcgaaagagatcaagagcgcgaacgcggcggaaattaccccgagccgtagcagcaacgaggaactggagaaagaactgaaccgttacgcgaaggcggttggtagcctggaaaccgcgtataaaccgtttctggcgagcagcgcgctggtgccgaccaccccgaccgcgttccaaaacgagctgaaaacctttcgtgacagcctgatcagcagctgcaagaaaaagaacatcctgattaccgataccagcagctggctgggcttccaggtttacagcacccaagcgccgagcgtgcaggcggcgagcaccctgggttttgagctgaaagcgattaacagcctggttaacaagctggcggaatgcggcctgagcaaattcatcaaggtgtatcgtccgcagctgccgattgaaaccccggcgaacaacccggaggaaagcgacgaagcggatcaggcgccgtggaccccgatgccgctggagatcgcgttccagggtgaccgtgaaagcgttctgaaagcgatgaacgcgattaccggcatgcaagattacctgtttaccgtgaacagcatccgtattcgtaacgaacgtatgatgccgccgccaatcgcgaacccggctgcggcgaagccggctgcggcgcagccggcgaccggtgcggcgagcctgaccccggcggacgaggctgcggcgccggctgcgccggcgatccagcaagttattaaaccgtatatgggcaaggaacaggtgttcgttcaagtgagcctgaacctggtgcactttaaccagccgaaagcgcaagagccgagcgaagattgacgagctcgatagtgctagtgtagatcgctactagagccaggcatcaaataaaacgaaaggctcagtcgaaagactgggcctttcgttttatctgttgtttgtcggtgaacgctctctactagagtcacactggctcaccttcgggtgggcctttctgcgtttatatactagaagcggccgctgcag

SEQ ID NO: 143 - DNA, 1288 bp, synthetic construct
  source 1..1288: mol_type = other DNA
tctagagcttgtcgacgtctcgagaaaaacgccgcaaagtttgagcgaagtcaataaactctctacccattcagggcaatatctctcttctcgaggaaagaggagaaagaagcttatgaagaaaaagatcattagcgcgatcctgatgagcaccgtgattctgagcgcggcggcgccgctgagcggtgtttatgcgggtagcagccatcatcaccaccaccacgacgacgacgacaaaattgttaacagcaagcgtagcgagctggataagaaaatcagcattgcggcgaaagagatcaagagcgcgaacgcggcggaaattaccccgagccgtagcagcaacgaggaactggagaaagaactgaaccgttacgcgaaggcggttggtagcctggaaaccgcgtataaaccgtttctggcgagcagcgcgctggtgccgaccaccccgaccgcgttccaaaacgagctgaaaacctttcgtgacagcctgatcagcagctgcaagaaaaagaacatcctgattaccgataccagcagctggctgggcttccaggtttacagcacccaagcgccgagcgtgcaggcggcgagcaccctgggttttgagctgaaagcgattaacagcctggttaacaagctggcggaatgcggcctgagcaaattcatcaaggtgtatcgtccgcagctgccgattgaaaccccggcgaacaacccggaggaaagcgacgaagcggatcaggcgccgtggaccccgatgccgctggagatcgcgttccagggtgaccgtgaaagcgttctgaaagcgatgaacgcgattaccggcatgcaagattacctgtttaccgtgaacagcatccgtattcgtaacgaacgtatgatgccgccgccaatcgcgaacccggctgcggcgaagccggctgcggcgcagccggcgaccggtgcggcgagcctgaccccggcggacgaggctgcggcgccggctgcgccggcgatccagcaagttattaaaccgtatatgggcaaggaacaggtgttcgttcaagtgagcctgaacctggtgcactttaaccagccgaaagcgcaagagccgagcgaagattgacgagctcgatagtgctagtgtagatcgctactagagccaggcatcaaataaaacgaaaggctcagtcgaaagactgggcctttcgttttatctgttgtttgtcggtgaacgctctctactagagtcacactggctcaccttcgggtgggcctttctgcgtttatatactagaagcggccgctgcag

SEQ ID NO: 144 - DNA, 838 bp, synthetic construct
  source 1..838: mol_type = other DNA
tctagagcttgtcgacgtctcgagtttacagctagctcagtcctaggtattatgctagcctcgaggaaagaggagaaagaagcttatgaagaaaaagatcattagcgcgatcctgatgagcaccgtgattctgagcgcggcggcgccgctgagcggtgtttatgcgagcccgggtcagggtacccaaagcgaaaacagctgcacccacttcccgggcaacctgccgaacatgctgcgtgacctgcgtgatgcgttcagccgtgtgaaaaccttcttccagatgaaagaccaactggataacctgctgctgaaggagagcctgctggaggacttcaaaggttacctgggctgccaggcgctgagcgaaatgatccaattttatctggaggaagtgatgccgcaggcggagaaccaagacccggatattaaggcgcacgttaacagcctgggcgagaacctgaaaaccctgcgtctgcgtctgcgtcgttgccaccgtttcctgccgtgcgagaacaaaagcaaggcggtggaacaggttaagaacgcgtttaacaaactgcaagagaagggcatctataaagcgatgagcgaattcgatatctttattaactacatcgaggcgtatatgaccatgaaaattcgtaactagtaacgagctcgatagtgctagtgtagatcgctactagagccaggcatcaaataaaacgaaaggctcagtcgaaagactgggcctttcgttttatctgttgtttgtcggtgaacgctctctactagagtcacactggctcaccttcgggtgggcctttctgcgtttatatactagaagcggccgctgcag

SEQ ID NO: 145 - DNA, 838 bp, synthetic construct
  source 1..838: mol_type = other DNA
tctagagcttgtcgacgtctcgagtttacggctagctcagtcctaggtacaatgctagcctcgaggaaagaggagaaagaagcttatgaagaaaaagatcattagcgcgatcctgatgagcaccgtgattctgagcgcggcggcgccgctgagcggtgtttatgcgagcccgggtcagggtacccaaagcgaaaacagctgcacccacttcccgggcaacctgccgaacatgctgcgtgacctgcgtgatgcgttcagccgtgtgaaaaccttcttccagatgaaagaccaactggataacctgctgctgaaggagagcctgctggaggacttcaaaggttacctgggctgccaggcgctgagcgaaatgatccaattttatctggaggaagtgatgccgcaggcggagaaccaagacccggatattaaggcgcacgttaacagcctgggcgagaacctgaaaaccctgcgtctgcgtctgcgtcgttgccaccgtttcctgccgtgcgagaacaaaagcaaggcggtggaacaggttaagaacgcgtttaacaaactgcaagagaagggcatctataaagcgatgagcgaattcgatatctttattaactacatcgaggcgtatatgaccatgaaaattcgtaactagtaacgagctcgatagtgctagtgtagatcgctactagagccaggcatcaaataaaacgaaaggctcagtcgaaagactgggcctttcgttttatctgttgtttgtcggtgaacgctctctactagagtcacactggctcaccttcgggtgggcctttctgcgtttatatactagaagcggccgctgcag

SEQ ID NO: 146 - DNA, 838 bp, synthetic construct
  source 1..838: mol_type = other DNA
tctagagcttgtcgacgtctcgagctgacagctagctcagtcctaggtataatgctagcctcgaggaaagaggagaaagaagcttatgaagaaaaagatcattagcgcgatcctgatgagcaccgtgattctgagcgcggcggcgccgctgagcggtgtttatgcgagcccgggtcagggtacccaaagcgaaaacagctgcacccacttcccgggcaacctgccgaacatgctgcgtgacctgcgtgatgcgttcagccgtgtgaaaaccttcttccagatgaaagaccaactggataacctgctgctgaaggagagcctgctggaggacttcaaaggttacctgggctgccaggcgctgagcgaaatgatccaattttatctggaggaagtgatgccgcaggcggagaaccaagacccggatattaaggcgcacgttaacagcctgggcgagaacctgaaaaccctgcgtctgcgtctgcgtcgttgccaccgtttcctgccgtgcgagaacaaaagcaaggcggtggaacaggttaagaacgcgtttaacaaactgcaagagaagggcatctataaagcgatgagcgaattcgatatctttattaactacatcgaggcgtatatgaccatgaaaattcgtaactagtaacgagctcgatagtgctagtgtagatcgctactagagccaggcatcaaataaaacgaaaggctcagtcgaaagactgggcctttcgttttatctgttgtttgtcggtgaacgctctctactagagtcacactggctcaccttcgggtgggcctttctgcgtttatatactagaagcggccgctgcag

SEQ ID NO: 147 - DNA, 814 bp, synthetic construct
  source 1..814: mol_type = other DNA
tctagagcttgtcgacgtctcgagtttacagctagctcagtcctaggtattatgctagcctcgaggaaagaggagaaagaagcttatgaagaaaatctggctggcgctggcgggtctggtgctggcgttcagcgcgagcgcgagcccgggtcagggtacccaaagcgaaaacagctgcacccacttcccgggcaacctgccgaacatgctgcgtgacctgcgtgatgcgttcagccgtgtgaaaaccttcttccagatgaaagaccaactggataacctgctgctgaaggagagcctgctggaggacttcaaaggttacctgggctgccaggcgctgagcgaaatgatccaattttatctggaggaagtgatgccgcaggcggagaaccaagacccggatattaaggcgcacgttaacagcctgggcgagaacctgaaaaccctgcgtctgcgtctgcgtcgttgccaccgtttcctgccgtgcgagaacaaaagcaaggcggtggaacaggttaagaacgcgtttaacaaactgcaagagaagggcatctataaagcgatgagcgaattcgatatctttattaactacatcgaggcgtatatgaccatgaaaattcgtaactagtaacgagctcgatagtgctagtgtagatcgctactagagccaggcatcaaataaaacgaaaggctcagtcgaaagactgggcctttcgttttatctgttgtttgtcggtgaacgctctctactagagtcacactggctcaccttcgggtgggcctttctgcgtttatatactagaagcggccgctgcag

SEQ ID NO: 148 - DNA, 820 bp, synthetic construct
  source 1..820: mol_type = other DNA
tctagagcttgtcgacgtctcgagtttacagctagctcagtcctaggtattatgctagcctcgaggaaagaggagaaagaagcttatgaagaaaaccgcgattgcgattgcggtggcgctggcgggtttcgcgaccgttgcgcaggcgagcccgggtcagggtacccaaagcgaaaacagctgcacccacttcccgggcaacctgccgaacatgctgcgtgacctgcgtgatgcgttcagccgtgtgaaaaccttcttccagatgaaagaccaactggataacctgctgctgaaggagagcctgctggaggacttcaaaggttacctgggctgccaggcgctgagcgaaatgatccaattttatctggaggaagtgatgccgcaggcggagaaccaagacccggatattaaggcgcacgttaacagcctgggcgagaacctgaaaaccctgcgtctgcgtctgcgtcgttgccaccgtttcctgccgtgcgagaacaaaagcaaggcggtggaacaggttaagaacgcgtttaacaaactgcaagagaagggcatctataaagcgatgagcgaattcgatatctttattaactacatcgaggcgtatatgaccatgaaaattcgtaactagtaacgagctcgatagtgctagtgtagatcgctactagagccaggcatcaaataaaacgaaaggctcagtcgaaagactgggcctttcgttttatctgttgtttgtcggtgaacgctctctactagagtcacactggctcaccttcgggtgggcctttctgcgtttatatactagaagcggccgctgcag

SEQ ID NO: 149 - DNA, 823 bp, synthetic construct
  source 1..823: mol_type = other DNA
tctagagcttgtcgacgtctcgagtttacagctagctcagtcctaggtattatgctagcctcgaggaaagaggagaaagaagcttatgaagtacctgctgccgaccgcggcggcgggtctgctgctgctggcggcgcagccggcgatggcgagcccgggtcagggtacccaaagcgaaaacagctgcacccacttcccgggcaacctgccgaacatgctgcgtgacctgcgtgatgcgttcagccgtgtgaaaaccttcttccagatgaaagaccaactggataacctgctgctgaaggagagcctgctggaggacttcaaaggttacctgggctgccaggcgctgagcgaaatgatccaattttatctggaggaagtgatgccgcaggcggagaaccaagacccggatattaaggcgcacgttaacagcctgggcgagaacctgaaaaccctgcgtctgcgtctgcgtcgttgccaccgtttcctgccgtgcgagaacaaaagcaaggcggtggaacaggttaagaacgcgtttaacaaactgcaagagaagggcatctataaagcgatgagcgaattcgatatctttattaactacatcgaggcgtatatgaccatgaaaattcgtaactagtaacgagctcgatagtgctagtgtagatcgctactagagccaggcatcaaataaaacgaaaggctcagtcgaaagactgggcctttcgttttatctgttgtttgtcggtgaacgctctctactagagtcacactggctcaccttcgggtgggcctttctgcgtttatatactagaagcggccgctgcag

SEQ ID NO: 150 - DNA, 1144 bp, synthetic construct
  source 1..1144: mol_type = other DNA
tctagagcttgtcgacgtctcgagtttacagctagctcagtcctaggtattatgctagcctcgaggaaagaggagaaagaagcttatgaaaaaaagaggggcgtttttagggctgttgttggtttctgcctgcgcatcagttttcgctgccaataatgaaaccagcaagtcggtcactttcccaaagtgtgaaggtctggatgctgccggaattgccgcgagcgtaaaacgtgattaccaacaaaatcgcgtggcgcgctgggctgatgatcaaaaaattgtcggtcaggccgatcccgtggcatgggtcagtttgcaggacattcaggggaaagatgataaatggtcagtaccgctaaccgtgcgtggtaaaagtgccgatattcattaccaggtcagcgtggactgcaaagcgggaatggcggaatatcagcggcgtcaccaccaccaccaccacgacgatgacgataagagcccgggtcagggtacccaaagcgaaaacagctgcacccacttcccgggcaacctgccgaacatgctgcgtgacctgcgtgatgcgttcagccgtgtgaaaaccttcttccagatgaaagaccaactggataacctgctgctgaaggagagcctgctggaggacttcaaaggttacctgggctgccaggcgctgagcgaaatgatccaattttatctggaggaagtgatgccgcaggcggagaaccaagacccggatattaaggcgcacgttaacagcctgggcgagaacctgaaaaccctgcgtctgcgtctgcgtcgttgccaccgtttcctgccgtgcgagaacaaaagcaaggcggtggaacaggttaagaacgcgtttaacaaactgcaagagaagggcatctataaagcgatgagcgaattcgatatctttattaactacatcgaggcgtatatgaccatgaaaattcgtaactagtaacgagctcgatagtgctagtgtagatcgctactagagccaggcatcaaataaaacgaaaggctcagtcgaaagactgggcctttcgttttatctgttgtttgtcggtgaacgctctctactagagtcacactggctcaccttcgggtgggcctttctgcgtttatatactagaagcggccgctgcag

SEQ ID NO: 151 - DNA, 847 bp, synthetic construct
  source 1..847: mol_type = other DNA
tctagagcttgtcgacgtctcgagtttacggctagctcagtcctaggtacaatgctagcctcgagttaagtttagaaagaggagaaagaagcttatgaagaaaaagatcattagcgcgatcctgatgagcaccgtgattctgagcgcggcggcgccgctgagcggtgtttatgcgagcccgggtcagggtacccaaagcgaaaacagctgcacccacttcccgggcaacctgccgaacatgctgcgtgacctgcgtgatgcgttcagccgtgtgaaaaccttcttccagatgaaagaccaactggataacctgctgctgaaggagagcctgctggaggacttcaaaggttacctgggctgccaggcgctgagcgaaatgatccaattttatctggaggaagtgatgccgcaggcggagaaccaagacccggatattaaggcgcacgttaacagcctgggcgagaacctgaaaaccctgcgtctgcgtctgcgtcgttgccaccgtttcctgccgtgcgagaacaaaagcaaggcggtggaacaggttaagaacgcgtttaacaaactgcaagagaagggcatctataaagcgatgagcgaattcgatatctttattaactacatcgaggcgtatatgaccatgaaaattcgtaactagtaacgagctcgatagtgctagtgtagatcgctactagagccaggcatcaaataaaacgaaaggctcagtcgaaagactgggcctttcgttttatctgttgtttgtcggtgaacgctctctactagagtcacactggctcaccttcgggtgggcctttctgcgtttatatactagaagcggccgctgcag

SEQ ID NO: 152 - DNA, 891 bp, synthetic construct
  source 1..891: mol_type = other DNA
tctagagcttgtcgacgtctcgagtttacggctagctcagtcctaggtacaatgctagcctcgaggaaagaggagaaagaagcttatgaaagcaattttcgtactgaaacatcttaatcatgctaaggaggttttctaatgaagaaaaagatcattagcgcgatcctgatgagcaccgtgattctgagcgcggcggcgccgctgagcggtgtttatgcgagcccgggtcagggtacccaaagcgaaaacagctgcacccacttcccgggcaacctgccgaacatgctgcgtgacctgcgtgatgcgttcagccgtgtgaaaaccttcttccagatgaaagaccaactggataacctgctgctgaaggagagcctgctggaggacttcaaaggttacctgggctgccaggcgctgagcgaaatgatccaattttatctggaggaagtgatgccgcaggcggagaaccaagacccggatattaaggcgcacgttaacagcctgggcgagaacctgaaaaccctgcgtctgcgtctgcgtcgttgccaccgtttcctgccgtgcgagaacaaaagcaaggcggtggaacaggttaagaacgcgtttaacaaactgcaagagaagggcatctataaagcgatgagcgaattcgatatctttattaactacatcgaggcgtatatgaccatgaaaattcgtaactagtaacgagctcgatagtgctagtgtagatcgctactagagccaggcatcaaataaaacgaaaggctcagtcgaaagactgggcctttcgttttatctgttgtttgtcggtgaacgctctctactagagtcacactggctcaccttcgggtgggcctttctgcgtttatatactagaagcggccgctgcag

SEQ ID NO: 153 - DNA, 870 bp, synthetic construct
  source 1..870: mol_type = other DNA
tctagagcttgtcgacgtctcgagtttacggctagctcagtcctaggtacaatgctagcctcgaggaaagaggagaaagaagcttatgcgtaaaggcgaagagaaggaggttaactgatgaagaaaaagatcattagcgcgatcctgatgagcaccgtgattctgagcgcggcggcgccgctgagcggtgtttatgcgagcccgggtcagggtacccaaagcgaaaacagctgcacccacttcccgggcaacctgccgaacatgctgcgtgacctgcgtgatgcgttcagccgtgtgaaaaccttcttccagatgaaagaccaactggataacctgctgctgaaggagagcctgctggaggacttcaaaggttacctgggctgccaggcgctgagcgaaatgatccaattttatctggaggaagtgatgccgcaggcggagaaccaagacccggatattaaggcgcacgttaacagcctgggcgagaacctgaaaaccctgcgtctgcgtctgcgtcgttgccaccgtttcctgccgtgcgagaacaaaagcaaggcggtggaacaggttaagaacgcgtttaacaaactgcaagagaagggcatctataaagcgatgagcgaattcgatatctttattaactacatcgaggcgtatatgaccatgaaaattcgtaactagtaacgagctcgatagtgctagtgtagatcgctactagagccaggcatcaaataaaacgaaaggctcagtcgaaagactgggcctttcgttttatctgttgtttgtcggtgaacgctctctactagagtcacactggctcaccttcgggtgggcctttctgcgtttatatactagaagcggccgctgcag

SEQ ID NO: 154 - DNA, 870 bp, synthetic construct
  source 1..870: mol_type = other DNA
tctagagcttgtcgacgtctcgagtttacggctagctcagtcctaggtacaatgctagcctcgaggaaagaggagaaagaagcttatgattatgtccggttataaggaggttaactgatgaagaaaaagatcattagcgcgatcctgatgagcaccgtgattctgagcgcggcggcgccgctgagcggtgtttatgcgagcccgggtcagggtacccaaagcgaaaacagctgcacccacttcccgggcaacctgccgaacatgctgcgtgacctgcgtgatgcgttcagccgtgtgaaaaccttcttccagatgaaagaccaactggataacctgctgctgaaggagagcctgctggaggacttcaaaggttacctgggctgccaggcgctgagcgaaatgatccaattttatctggaggaagtgatgccgcaggcggagaaccaagacccggatattaaggcgcacgttaacagcctgggcgagaacctgaaaaccctgcgtctgcgtctgcgtcgttgccaccgtttcctgccgtgcgagaacaaaagcaaggcggtggaacaggttaagaacgcgtttaacaaactgcaagagaagggcatctataaagcgatgagcgaattcgatatctttattaactacatcgaggcgtatatgaccatgaaaattcgtaactagtaacgagctcgatagtgctagtgtagatcgctactagagccaggcatcaaataaaacgaaaggctcagtcgaaagactgggcctttcgttttatctgttgtttgtcggtgaacgctctctactagagtcacactggctcaccttcgggtgggcctttctgcgtttatatactagaagcggccgctgcag

SEQ ID NO: 155 - DNA, 921 bp, synthetic construct
  source 1..921: mol_type = other DNA
tctagagcttgtcgacgtctcgagaaaaacgccgcaaagtttgagcgaagtcaataaactctctacccattcagggcaatatctctcttctcgaggaaagaggagaaagaagcttatgaaagcaattttcgtactgaaacatcttaatcatgctaaggaggttttctaatgaagaaaaagatcattagcgcgatcctgatgagcaccgtgattctgagcgcggcggcgccgctgagcggtgtttatgcgagcccgggtcagggtacccaaagcgaaaacagctgcacccacttcccgggcaacctgccgaacatgctgcgtgacctgcgtgatgcgttcagccgtgtgaaaaccttcttccagatgaaagaccaactggataacctgctgctgaaggagagcctgctggaggacttcaaaggttacctgggctgccaggcgctgagcgaaatgatccaattttatctggaggaagtgatgccgcaggcggagaaccaagacccggatattaaggcgcacgttaacagcctgggcgagaacctgaaaaccctgcgtctgcgtctgcgtcgttgccaccgtttcctgccgtgcgagaacaaaagcaaggcggtggaacaggttaagaacgcgtttaacaaactgcaagagaagggcatctataaagcgatgagcgaattcgatatctttattaactacatcgaggcgtatatgaccatgaaaattcgtaactagtaacgagctcgatagtgctagtgtagatcgctactagagccaggcatcaaataaaacgaaaggctcagtcgaaagactgggcctttcgttttatctgttgtttgtcggtgaacgctctctactagagtcacactggctcaccttcgggtgggcctttctgcgtttatatactagaagcggccgctgcag

SEQ ID NO: 156 - DNA, 868 bp, synthetic construct
  source 1..868: mol_type = other DNA
tctagagcttgtcgacgtctcgagaaaaacgccgcaaagtttgagcgaagtcaataaactctctacccattcagggcaatatctctcttctcgaggaaagaggagaaagaagcttatgaagaaaaagatcattagcgcgatcctgatgagcaccgtgattctgagcgcggcggcgccgctgagcggtgtttatgcgagcccgggtcagggtacccaaagcgaaaacagctgcacccacttcccgggcaacctgccgaacatgctgcgtgacctgcgtgatgcgttcagccgtgtgaaaaccttcttccagatgaaagaccaactggataacctgctgctgaaggagagcctgctggaggacttcaaaggttacctgggctgccaggcgctgagcgaaatgatccaattttatctggaggaagtgatgccgcaggcggagaaccaagacccggatattaaggcgcacgttaacagcctgggcgagaacctgaaaaccctgcgtctgcgtctgcgtcgttgccaccgtttcctgccgtgcgagaacaaaagcaaggcggtggaacaggttaagaacgcgtttaacaaactgcaagagaagggcatctataaagcgatgagcgaattcgatatctttattaactacatcgaggcgtatatgaccatgaaaattcgtaactagtaacgagctcgatagtgctagtgtagatcgctactagagccaggcatcaaataaaacgaaaggctcagtcgaaagactgggcctttcgttttatctgttgtttgtcggtgaacgctctctactagagtcacactggctcaccttcgggtgggcctttctgcgtttatatactagaagcggccgctgcag

SEQ ID NO: 157 - DNA, 786 bp, synthetic construct
  source 1..786: mol_type = other DNA
tctagagtctcgagttgacagctagctcagtcctaggtataatgctagcctcgaggaaagaggagaaagaagcttatgaagaaaaagatcattagcgcgatcctgatgagcaccgtgattctgagcgcggcggcgccgctgagcggtgtttatgcggcgccgatcagcagccactgccgtctggacaaaagcaacttccagcaaccgtatattaccaaccgtacctttatgctggcgaaagaggcgagcctggcggacaacaacaccgatgtgcgtctgatcggcgagaaactgttccacggcgttagcatgagcgaacgttgctacctgatgaagcaggtgctgaactttaccctggaggaagttctgttcccgcaaagcgatcgttttcagccgtatatgcaagaggtggttccgttcctggcgcgtctgagcaaccgtctgagcacctgccacatcgaaggtgacgatctgcacattcagcgtaacgtgcaaaaactgaaggacaccgttaaaaagctgggcgagagcggcgaaatcaaagcgattggcgaactggatctgctgtttatgagcctgcgtaacgcgtgcatttagtaacgagctcgatagtgctagtgtagatcgctactagagccaggcatcaaataaaacgaaaggctcagtcgaaagactgggcctttcgttttatctgttgtttgtcggtgaacgctctctactagagtcacactggctcaccttcgggtgggcctttctgcgtttatatactagaagcggccgctgcag

SEQ ID NO: 158 - DNA, 796 bp, synthetic construct
  source 1..796: mol_type = other DNA
tctagagcttgtcgacgtctcgagtttacagctagctcagtcctaggtattatgctagcctcgaggaaagaggagaaagaagcttatgaagaaaaagatcattagcgcgatcctgatgagcaccgtgattctgagcgcggcggcgccgctgagcggtgtttatgcggcgccgatcagcagccactgccgtctggacaaaagcaacttccagcaaccgtatattaccaaccgtacctttatgctggcgaaagaggcgagcctggcggacaacaacaccgatgtgcgtctgatcggcgagaaactgttccacggcgttagcatgagcgaacgttgctacctgatgaagcaggtgctgaactttaccctggaggaagttctgttcccgcaaagcgatcgttttcagccgtatatgcaagaggtggttccgttcctggcgcgtctgagcaaccgtctgagcacctgccacatcgaaggtgacgatctgcacattcagcgtaacgtgcaaaaactgaaggacaccgttaaaaagctgggcgagagcggcgaaatcaaagcgattggcgaactggatctgctgtttatgagcctgcgtaacgcgtgcatttagtaacgagctcgatagtgctagtgtagatcgctactagagccaggcatcaaataaaacgaaaggctcagtcgaaagactgggcctttcgttttatctgttgtttgtcggtgaacgctctctactagagtcacactggctcaccttcgggtgggcctttctgcgtttatatactagaagcggccgctgcag

SEQ ID NO: 159 - DNA, 796 bp, synthetic construct
  source 1..796: mol_type = other DNA
tctagagcttgtcgacgtctcgagttgacagctagctcagtcctaggtactgtgctagcctcgaggaaagaggagaaagaagcttatgaagaaaaagatcattagcgcgatcctgatgagcaccgtgattctgagcgcggcggcgccgctgagcggtgtttatgcggcgccgatcagcagccactgccgtctggacaaaagcaacttccagcaaccgtatattaccaaccgtacctttatgctggcgaaagaggcgagcctggcggacaacaacaccgatgtgcgtctgatcggcgagaaactgttccacggcgttagcatgagcgaacgttgctacctgatgaagcaggtgctgaactttaccctggaggaagttctgttcccgcaaagcgatcgttttcagccgtatatgcaagaggtggttccgttcctggcgcgtctgagcaaccgtctgagcacctgccacatcgaaggtgacgatctgcacattcagcgtaacgtgcaaaaactgaaggacaccgttaaaaagctgggcgagagcggcgaaatcaaagcgattggcgaactggatctgctgtttatgagcctgcgtaacgcgtgcatttagtaacgagctcgatagtgctagtgtagatcgctactagagccaggcatcaaataaaacgaaaggctcagtcgaaagactgggcctttcgttttatctgttgtttgtcggtgaacgctctctactagagtcacactggctcaccttcgggtgggcctttctgcgtttatatactagaagcggccgctgcag

SEQ ID NO: 160 - DNA, 796 bp, synthetic construct
  source 1..796: mol_type = other DNA
tctagagcttgtcgacgtctcgagctgacagctagctcagtcctaggtataatgctagcctcgaggaaagaggagaaagaagcttatgaagaaaaagatcattagcgcgatcctgatgagcaccgtgattctgagcgcggcggcgccgctgagcggtgtttatgcggcgccgatcagcagccactgccgtctggacaaaagcaacttccagcaaccgtatattaccaaccgtacctttatgctggcgaaagaggcgagcctggcggacaacaacaccgatgtgcgtctgatcggcgagaaactgttccacggcgttagcatgagcgaacgttgctacctgatgaagcaggtgctgaactttaccctggaggaagttctgttcccgcaaagcgatcgttttcagccgtatatgcaagaggtggttccgttcctggcgcgtctgagcaaccgtctgagcacctgccacatcgaaggtgacgatctgcacattcagcgtaacgtgcaaaaactgaaggacaccgttaaaaagctgggcgagagcggcgaaatcaaagcgattggcgaactggatctgctgtttatgagcctgcgtaacgcgtgcatttagtaacgagctcgatagtgctagtgtagatcgctactagagccaggcatcaaataaaacgaaaggctcagtcgaaagactgggcctttcgttttatctgttgtttgtcggtgaacgctctctactagagtcacactggctcaccttcgggtgggcctttctgcgtttatatactagaagcggccgctgcag

SEQ ID NO: 161 - DNA, 796 bp, synthetic construct
  source 1..796: mol_type = other DNA
tctagagcttgtcgacgtctcgagtttacggctagctcagtcctaggtacaatgctagcctcgaggaaagaggagaaagaagcttatgaagaaaaagatcattagcgcgatcctgatgagcaccgtgattctgagcgcggcggcgccgctgagcggtgtttatgcggcgccgatcagcagccactgccgtctggacaaaagcaacttccagcaaccgtatattaccaaccgtacctttatgctggcgaaagaggcgagcctggcggacaacaacaccgatgtgcgtctgatcggcgagaaactgttccacggcgttagcatgagcgaacgttgctacctgatgaagcaggtgctgaactttaccctggaggaagttctgttcccgcaaagcgatcgttttcagccgtatatgcaagaggtggttccgttcctggcgcgtctgagcaaccgtctgagcacctgccacatcgaaggtgacgatctgcacattcagcgtaacgtgcaaaaactgaaggacaccgttaaaaagctgggcgagagcggcgaaatcaaagcgattggcgaactggatctgctgtttatgagcctgcgtaacgcgtgcatttagtaacgagctcgatagtgctagtgtagatcgctactagagccaggcatcaaataaaacgaaaggctcagtcgaaagactgggcctttcgttttatctgttgtttgtcggtgaacgctctctactagagtcacactggctcaccttcgggtgggcctttctgcgtttatatactagaagcggccgctgcag

SEQ ID NO: 162 - DNA, 796 bp, synthetic construct
  source 1..796: mol_type = other DNA
tctagagcttgtcgacgtctcgagtttatggctagctcagtcctaggtacaatgctagcctcgaggaaagaggagaaagaagcttatgaagaaaaagatcattagcgcgatcctgatgagcaccgtgattctgagcgcggcggcgccgctgagcggtgtttatgcggcgccgatcagcagccactgccgtctggacaaaagcaacttccagcaaccgtatattaccaaccgtacctttatgctggcgaaagaggcgagcctggcggacaacaacaccgatgtgcgtctgatcggcgagaaactgttccacggcgttagcatgagcgaacgttgctacctgatgaagcaggtgctgaactttaccctggaggaagttctgttcccgcaaagcgatcgttttcagccgtatatgcaagaggtggttccgttcctggcgcgtctgagcaaccgtctgagcacctgccacatcgaaggtgacgatctgcacattcagcgtaacgtgcaaaaactgaaggacaccgttaaaaagctgggcgagagcggcgaaatcaaagcgattggcgaactggatctgctgtttatgagcctgcgtaacgcgtgcatttagtaacgagctcgatagtgctagtgtagatcgctactagagccaggcatcaaataaaacgaaaggctcagtcgaaagactgggcctttcgttttatctgttgtttgtcggtgaacgctctctactagagtcacactggctcaccttcgggtgggcctttctgcgtttatatactagaagcggccgctgcag

SEQ ID NO: 163 - DNA, 826 bp, synthetic construct
  source 1..826: mol_type = other DNA
tctagagcttgtcgacgtctcgagaaaaacgccgcaaagtttgagcgaagtcaataaactctctacccattcagggcaatatctctcttctcgaggaaagaggagaaagaagcttatgaagaaaaagatcattagcgcgatcctgatgagcaccgtgattctgagcgcggcggcgccgctgagcggtgtttatgcggcgccgatcagcagccactgccgtctggacaaaagcaacttccagcaaccgtatattaccaaccgtacctttatgctggcgaaagaggcgagcctggcggacaacaacaccgatgtgcgtctgatcggcgagaaactgttccacggcgttagcatgagcgaacgttgctacctgatgaagcaggtgctgaactttaccctggaggaagttctgttcccgcaaagcgatcgttttcagccgtatatgcaagaggtggttccgttcctggcgcgtctgagcaaccgtctgagcacctgccacatcgaaggtgacgatctgcacattcagcgtaacgtgcaaaaactgaaggacaccgttaaaaagctgggcgagagcggcgaaatcaaagcgattggcgaactggatctgctgtttatgagcctgcgtaacgcgtgcatttagtaacgagctcgatagtgctagtgtagatcgctactagagccaggcatcaaataaaacgaaaggctcagtcgaaagactgggcctttcgttttatctgttgtttgtcggtgaacgctctctactagagtcacactggctcaccttcgggtgggcctttctgcgtttatatactagaagcggccgctgcag

SEQ ID NO: 164 - DNA, 20 bp, synthetic construct
  source 1..20: mol_type = other DNA
gctgccgctattctgccgct

SEQ ID NO: 165 - DNA, 20 bp, synthetic construct
  source 1..20: mol_type = other DNA
atgaaggagaaaactcaccg

SEQ ID NO: 166 - DNA, 20 bp, synthetic construct
  source 1..20: mol_type = other DNA
gggaaacgggataatctgag

SEQ ID NO: 167 - DNA, 405 bp, synthetic construct
  source 1..405: mol_type = other DNA
gtgaatacaacgctgtttcgatggccggttcgtgtctactatgaagataccgatgccggtggtgtggtgtaccacgccagttacgtcgctttttatgaaagagcacgcacagagatgctgcgtcatcatcatttcagtcaacaggcgctgatggctgaacgcgttgcctttgtggtacgtaaaatgacggtggaatattacgcacctgcgcggctcgacgatatgctcgaaatacagactgaaataacatcaatgcgtggcacctctttggttttcacgcaacgtattgtcaacgccgagaatactttgttgaatgaagcagaggttctggttgtttgcgttgacccactcaaaatgaagcctcgtgcgcttcccaagtctattgtcgcggagtttaagcagtga

SEQ ID NO: 168 - DNA, 496 bp, synthetic construct
  source 1..496: mol_type = other DNA
gccatggccagagcgcgtggacgaggtcgtcgcgatctcaagtccgaaatcaacattgtaccgttgctggacgtactgctggtgctgttgctgatctttatggcgacagcgcccatcatcacccagagcgtggaggtcgatctgccagacgctactgaatcacaggcggtgagcagtaacgataatccgccagtgattgttgaagtgtctggtattggtcagtacaccgtggtggttgagaaagatcgtctggagcgtttaccaccagagcaggtggtggcggaagtgtccagccgtttcaaggccaacccgaaaacggtctttctgatcggtggcgcaaaagatgtgccttacgatgaaataattaaagcactgaacttgttacatagtgcgggtgtgaaatcggttggtttaatgacgcagcctatctaaacatctgcgtttcccttgcttgaaagagagcgggtaacaggcgaacagtttttggaaaccgaga

SEQ ID NO: 169 - DNA, 20 bp, synthetic construct
  source 1..20: mol_type = other DNA
tggtattggtcagtacaccg

SEQ ID NO: 170 - DNA, 415 bp, synthetic construct
  source 1..415: mol_type = other DNA
gcatcgtgccaatagccatgcgccggaagccgtagtggaaggggcgtcgcgtgcgatgcgtatttccatgaatcgtgaacttgaaaatctggaaacgcacattcctttcctcggtacggttggctccatcagcccgtatattggtctgtttggtacggtctgggggatcatgcacgcctttatcgccctcggggcggtaaaacaagcaacactgcaaatggttgcgcccggtatcgcagaagcgttgattgcgacggcaattggtttgttcgccgcaattccggcggtaatggcttataaccgcctcaaccagcgcgtaaacaaactggaactgaattacgacaactttatggaagagtttaccgcgattctgcaccgccaggcgtttaccgttagcgagagcaacaaggggtaa

SEQ ID NO: 171 - DNA, 474 bp, synthetic construct
  source 1..474: mol_type = other DNA
acatctgcgtttcccttgcttgaaagagagcgggtaacaggcgaacagtttttggaaaccgagagtgtcaaaggcaaccgaacaaaacgacaagctcaagcgggcgataattatttcagcagtgctgcatgtcatcttatttgcggcgctgatctggagttcgttcgatgagaatatagaagcttcagccggaggcggcggtggttcgtccatcgacgctgtcatggttgattcaggtgcggtagttgaacagtacaaacgtatgcaaagccaggaatcaagcgcgaagcgttctgatgagcagcgcaagatgaaggagcagcaggctgctgaagaactgcgtgagaaacaagcggctgaacaggaacgcctgaagcaacttgagaaagagcggttagcggctcaggagcagaaaaagcaggctgaagaagccgcaaaacaggccgagttaaagcagaagcaagcggaagaggc

SEQ ID NO: 172 - DNA, 20 bp, synthetic construct
  source 1..20: mol_type = other DNA
agaactgcgtgagaaacaag

SEQ ID NO: 173 - DNA, 496 bp, synthetic construct; identical to SEQ ID NO: 168
  source 1..496: mol_type = other DNA

SEQ ID NO: 174 - DNA, 500 bp, synthetic construct
  source 1..500: mol_type = other DNA
tcgcgatgttgactgttccgacggtcaacatcaggcaccggttgccacggggttctggtagttttgtgtattttagtttgttaacattctgctaaattatcgtgggccatcggtccagataagggagatatgatgaagcaggcattacgagtagcatttggttttctcatactgtgggcatcagttctgcatgctgaagtccgcattgtgatcgacagcggtgtagattccggtcgtcctattggtgttgttcctttccagtgggcggggcctggtgcggcacctgaagatattggcggcatcgttgctgctgacttgcgtaacagcggtaaatttaatccgttagatcgtgctcgtttgccacagcagccgggtagtgcgcaggaagtacaaccagctgcatggtccgcgctgggcattgacgctgtggttgtcggtcaggtcactccgaatccggatggttcttacaatgttgcttatcaacttgttgacactggcgg

SEQ ID NO: 175 - DNA, 20 bp, synthetic construct
  source 1..20: mol_type = other DNA
agtcaccgtagaaggtcacg

SEQ ID NO: 176 - DNA, 473 bp, synthetic construct
  source 1..473: mol_type = other DNA
tggtcgcagtaacaataccgaaccgacctggttcccggacagccagaacctggcatttacttctgaccaggccggtcgtccgcaggtttataaagtgaatatcaacggcggtgcgccacaacgtattacctgggaaggttcgcagaaccaggatgcggatgtcagcagcgacggtaaatttatggtaatggtcagctccaacggtgggcagcagcacattgccaaacaagatctggcaacgggaggcgtacaagttctgtcgtccacgttcctggatgaaacgccaagtctggcacctaacggcactatggtaatctacagctcttctcaggggatgggatccgtgctgaatttggtttctacagatgggcgtttcaaagcgcgtcttccggcaactgatggacaggtcaaattccctgcctggtcgccgtatctgtgataataattaattgaatagtaaaggaatcattgaa

SEQ ID NO: 177 - DNA, 471 bp, synthetic construct
  source 1..471: mol_type = other DNA
gagaattgcatgagcagtaacttcagacatcaactattgagtctgtcgttactggttggtatagcggccccctgggccgcttttgctcaggcaccaatcagtagtgtcggctcaggctcggtcgaagaccgcgtcactcaacttgagcgtatttctaatgctcacagccagcttttaacccaactccagcaacaactctctgataatcaatccgatattgattccctgcgtggtcagattcaggaaaatcagtatcaactgaatcaggtcgtggagcggcaaaagcagatcctgttgcagatcgacagcctcagcagcggtggtgcagcggcgcaatcaaccagcggcgatcaaagcggtgtggcggcatcaacgacgccgacagctgatgctggtactgcgaatgctggcgcgccggtgaaaagcggtgatgcaaacacggattacaatgcagctattgcgctggtgcag

SEQ ID NO: 178 - DNA, 20 bp, synthetic construct
  source 1..20: mol_type = other DNA
acgttcaggctgctaaagat

SEQ ID NO: 179 - DNA, 482 bp, synthetic construct
  source 1..482: mol_type = other DNA
aatacttcccggatgccaccatcctggcactgaccaccaacgaaaaaacggctcaccagttagtactgagcaaaggtgttgtgccgcagctggttaaagagatcacatctactgatgacttctaccgtctgggtaaagaactggctctgcagagcggtctggcacacaaaggtgatgtcgtagttatggtttctggtgcactggtaccgagcggcactactaacaccgcatctgttcacgtcctgtaatattgcttttgtgaattaatttgtatatcgaagcgccctgatgggcgctttttttatttaatcgataaccagaagcaataaaaaatcaaatcggatttcactatataatctcactttatctaagatgaatccgatggaagcatcctgttttctctcaatttttttatctaaaacccagcgttcgatgcttctttgagcgaacgatcaaaaataagtgccttcccatcaaaaaaa

SEQ ID NO: 180 - DNA, 438 bp, synthetic construct
  source 1..438: mol_type = other DNA
cctgtgaagtgaaaaatggcgcacattgtgcgccatttttttgcctgctatttaccgctactgcgtcgcgcgtaacatattcccttgctctggttccccattctgcgctgactctactgaaggcgcattgctggctgcgggagttgctccactgctcaccgcaaccggataccctgcccgacgatacaacgctttatcgactaacttctgatctacagccttattgtctttaaattgcgtaaagcctgctggcagcgtgtacggcattgtctgaacgttctgctgttcttctgccgatagtggtcgatgtacttcaacataacgcatcccgttaggttccacggaatatttcaccggttcgttgatcactttcaccggtgttcccgtccgcacgctggagaataaagctttaatatccggtgcattcatgcgaataca

SEQ ID NO: 181 - DNA, 20 bp, synthetic construct
  source 1..20: mol_type = other DNA
caaaccgttcctctacaccg

SEQ ID NO: 182 - DNA, 417 bp, synthetic construct
  source 1..417: mol_type = other DNA
gacagccaggccatttgctcccgctcaccgagggacatcgacgggcgtggaaatgaccgctgtaatgtgcgactggcgggaaacgccaacataatgtgatgacgctgcggcagttcacgactccacggtaacaacgtgttagccagccgctgcacatcaacaatccgcccatctttgataatgtcgttctccagtggcaaccgccaccagcggtgcaataagcattcttttgcgctccgcacgatagcaaccgctaccgcttcttgctgttgtaaatgcaaaccaatttgccagttcttaaatgccattgtgatgatctccttatcacccgtcactctgacgggtatatcaatgcgtctggcttgcctttatactaccgcgcgtttgtttataaactgcccaaatgaaactaaatgg

SEQ ID NO: 183 - DNA, 460 bp, synthetic construct
  source 1..460: mol_type = other DNA
ttaaaaaggcgcttcggcgcctttttcagtttgctgacaaagtgcacttgtttatgccagatgcgggtgaacgcgttatccggccaacaaaaaattgaaaattcaataaattgcaggaacttcgtaagcctgataagcgttgtgcatcaggcaaacttcacgcatttacactcgcccctgccctttcaaccattcgcgcacgaggaacagcgcgctgacattacgcgcttcgttgaagtcaggggcttccagcaaatccatcatatgcgccagcggccagcgcacctgtggtagcggctctggctcatcgccttccagtgattccgggtagagatcttgcgctaccacgatattcattttgctggaaaagtaagacggtgccatgctgagcttcttcaaaaaagtcagatcgttcgcaccaaatccaacctcttcttttagctcgcggttagcggcttca

SEQ ID NO: 184 - DNA, 20 bp, synthetic construct
  source 1..20: mol_type = other DNA
cctgggactcatggccggat

SEQ ID NO: 185 - DNA, 516 bp, synthetic construct
  source 1..516: mol_type = other DNA
cccagcccttgtcgatgccgcgttcaggctagcttcgttcaaatccattaaagatatcagactactctcaggtacgtgagtaaggtaaaacccagttccaacgccaatatccagatggttgttacctaaatgttccagaaagtgtggaagaaggtgttcctttgtaggacatccccatgcaagccgatttgatactcccaaaacccaccagtcataaagctttagggtaagtggtgtgtaaattttagccccatcatctgtgttttttttcattagtttcaccgtgttatagttttatttgtgaattaaatcaattatagagatgaattacaaggggttaaatgatgccacggcataacgaatttgaatatattgggtcttgtgttgcggtaagaggttacacgccaggacgcaggttaaatgcttacaatattaggggatattgtttgcttttaacggtaaacaaattccccggggctatacaataccaccggggagaaaatctatttaacgttg

SEQ ID NO: 186 - DNA, 623 bp, synthetic construct
  source 1..623: mol_type = other DNA
aaaaggtctccattcaatcgttttaatgattgagtatgtattttttatatctaacttaatgagtcaattgtatattgccccactgtttatattttgtttaacattgaatttttgtcacaatgcgctgtcagttttttagtttaattgtctgtttgtgttttgtattgtggttttatgggctaattatttttttctttgtggagtttttatctattcaagtgccatgcctttagatgcatattagcgataatagcatgaggtttatcctcaattgctgtgttttttagtataaaaaagaggaacaaaactgagacacataaggcctcgcaatggcttgcaaggttttacatattttgaggtggtggaacgtgtgaacgcagagatggcgcggtaatttgttgatttaaaatgtcgttcttggagtttctaagtcgtgggctacaggttcgaatcctgcagggcgagccatttcctcgccatttatttgttcccttttacaaattacaccatcactttgttgtcgcggttttgctaaataattggaacacgtcagacgaataaaatgaaaacagaaattctgctaaacaattcatcttgccaggattttgattaggaaagtgaaa

SEQ ID NO: 187 - DNA, 1756 bp, synthetic construct
  source 1..1756: mol_type = other DNA
gaattccggatgagcattcatcaggcgggcaagaatgtgaataaaggccggataaaacttgtgcttatttttctttacggtctttaaaaaggccgtaatatccagctgaacggtctggttataggtacattgagcaactgactgaaatgcctcaaaatgttctttacgatgccattgggatatatcaacggtggtatatccagtgatttttttctccattttagcttccttagctcctgaaaatctcgataactcaaaaaatacgcccggtagtgatcttatttcattatggtgaaagttggaacctcttacgtgccgatcaacgtctcattttcgccaaaagttggcccagggcttcccggtatcaacagggacaccaggatttatttattctgcgaagtgatcttccgtcacaggtatttattcgggatcctcgctcactgactcgctacgctcggtcgttcgactgcggcgagcggaaatggcttacgaacggggcggagatttcctggaagatgccaggaagatacttaacagggaagtgagagggccgcggcaaagccgtttttccataggctccgcccccctgacaagcatcacgaaatctgacgctcaaatcagtggtggcgaaacccgacaggactataaagataccaggcgtttccccctggcggctccctcgtgcgctctcctgttcctgcctttcggtttaccggtgtcattccgctgttatggccgcgtttgtctcattccacgcctgacactcagttccgggtaggcagttcgctccaagctggactgtatgcacgaaccccccgttcagtccgaccgctgcgccttatccggtaactatcgtcttgagtccaacccggaaagacatgcaaaagcaccactggcagcagccactggtaattgatttagaggagttagtcttgaagtcatgcgccggttaaggctaaactgaaaggacaagttttggtgactgcgctcctccaagccagttacctcggttcaaagagttggtagctcagagaaccttcgaaaaaccgccctgcaaggcggttttttcgttttcagagcaagagattacgcgcagaccaaaacgatctcaagaagatcatctgtaggtcgttcgctccaagctggaaggatcttcacctagatccttttaaattaaaaatgaagttttaaatcaatctaaagtatatatgagtaaacttggtctgacagaatttctgccattcatccgcttattatcacttattcaggcgtagcaaccaggcgtttaagggcaccaataactgccttaaaaaaattacgccccgccctgccactcatcgcagtactgttgtaattcattaagcattctgccgacatggaagccatcacaaacggcatgatgaacctgaatcgccagcggcatcagcaccttgtcgccttgcgtataatatttgcccatggtgaaaacgggggcgaagaagttgtccatattggccacgtttaaatcaaaactggtgaaactcacccagggattggctgagacgaaaaacatattctcaataaaccctttagggaaataggccaggttttcaccgtaacacgccacatcttgcgaatatatgtgtagaaactgccggaaatcgtcgtggtattcactccagagcgatgaaaacgtttcagtttgctcatggaaaacggtgtaacaagggtgaacactatcccatatcaccagctcaccgtctttcattgccatacg

SEQ ID NO: 188 - DNA, 20 bp, synthetic construct
  source 1..20: mol_type = other DNA
gagggtgagccataatgaag

SEQ ID NO: 189 - DNA, 553 bp, synthetic construct
  source 1..553: mol_type = other DNA
tccgagacataaggcgcatccggtaatttatccagttgctggcgcagcataaaaatcagctcaaatacatgatcgggcagcgtaatttcaccaatctctttctgccagcgttcatattcttcatctgtgatctgcaaggaggcaggaaccggattgtcattttcatcctgttgactggtcagcatggagcggaaattcgctttatcctgcactttatctaaccacagacgaatcagcatgcgatcatataacgcttccagactgctgtctgcttccggcagctcgttggaggccgccaccagcagacgcatcgggattttttctacgagtgcgccgttgcggaactggcgctcgttaatggcggtgagcagggtattaagaattgccggacccgctttccagatctcatccagaaagacgatttcagcttccggcaggtaaccgctggttaaacgttcatagcgcccttcatcttttagcgcctgaatagaaaggggaccaaaaacttcttccggcgtggagaagcgggtcatcagatattcaaacgcgcggg

SEQ ID NO: 190 - DNA, 340 bp, synthetic construct
  source 1..340: mol_type = other DNA
aatgtggccgcatttaggagtacgattttgccgttaatcgtgcatactgtgcgcttttttgtgggccaagggactaagcacacatttcatatttcaacgaaagactagtctatgagcactgataataagcaatcattgcccgcgattaccctcgcggcgattggagttgtctacggcgatattggtaccagcccgttatatacacttcgtgaatgtttgtccggccagtttggttttggcgttgaacgcgatgccgtgtttggctttttatcgctgatcttctggctgctaatctttgtggtttccattaaatatctcaccttcgtgatgcgggcagata

SEQ ID NO: 191 - DNA, 20 bp, synthetic construct
  source 1..20: mol_type = other DNA
ctgaccaacgcttctttacc

SEQ ID NO: 192 - DNA, 473 bp, synthetic construct
  source 1..473: mol_type = other DNA
aacgaaacgctatcgataagaataaaaaggaataaaagtggaatataaagtctggcacttcttactgaccacgcaaacacctttcgtacagcatgatgagagcggcaaaagcaaactacacttatgcttcattcgatgcacatttgcagaaggttgccgctatgaagccaacgatgctactcatgattaccgtattcctgatttttccagccatttctcaggccgagtcgccattcagttctctacagtcggcaaaagagaaaaccacggtattgcaagatttacgtaaaatttgcacgccacaggcgtcattatcagatgaagcgtgggaaaagttaatgttgtcagatgaaaacaataaacaacatatacgcgaggccatcgtggcgatggaacgtaataatcagagcaattattgggaagcgttgggtaaggtagaatgcccggatatgtaagaacggcaacaaccactg

SEQ ID NO: 193 - DNA, 464 bp, synthetic construct
  source 1..464: mol_type = other DNA
accaacgcttctttacctgatatcaggatttcttcattttcacctttgcagtcaccaacaatgcagtcagcaacatcaatgtgccggacaacatcagcggcgaagtcagaccaatgttatccaacgcataaccgccgattgccgcaccgcaggtgttagcaagctgaataacggccacctgaatagatccagccttttctgcctgatcggccaatgagcgagtgatccacgttgaccaaccaacgggaattaaagcaaaggtcagcccccagataatcgcaacaccagtagcaacaattttatagcttccccacagcgtcagtaccagcgcgctcagggcgagcacaaacggtgcgcccgctaaggccagtttcaccgaacgtttgagaataaacgacgaaagcgatgtcccgacaaagctggcgataccaaaactcagcagcaccagggttaagccatcaaca

SEQ ID NO: 194 - DNA, 20 bp, synthetic construct
  source 1..20: mol_type = other DNA
gaaggggaagaggcgcgcgt

SEQ ID NO: 195 - DNA, 419 bp, synthetic construct
  source 1..419: mol_type = other DNA
gtggtggatgacggtaaacgtaccctcgatgatgtgattgaaggcgcggatattttcctcggctgttccggcccgaaagtgctgacccaggaaatggtgaagaaaatggcccgtgcgccaatgatcctggcgctggcgaacccggaaccggaaattctgccgccgctggcgaaagaagtgcgtccggatgccatcatctgtaccggccgttccgactacccgaaccaggtgaacaacgtcctttgcttcccgtttatcttccgtggcgcgctggacgttggcgcaaccgccatcaacgaagagatgaaactggcggcagtacgcgcgattgcagaactggcccatgcggaacagagtgaagtggtggcttcagcgtatggcgatcaggatctgagctttggtccggaatacatcattcc

SEQ ID NO: 196 - DNA, 347 bp, synthetic construct
  source 1..347: mol_type = other DNA
gcgaaaccgatccttattggtcgtccgaacgtgatcgaaatgcgcattcagaaactgggcttgcagatcaagtcgggcgttgattttgagatcgtcaataacgaatccgatccgcgctttaaagagtactggaccgaatacttccagatcatgaagcgtcgcggtgtcactcaggagcaggcgcagcgtgcgctgatcagtaacccgacagtgatcggcgcgatcatggttcagcgtggcgaagccgatgcaatgatttgcggtacggtgggcgattatcatgaacactttagcgtggtgaaaaatgtctttggttatcgcgatggcgttcacaccgcaggtgcaat

SEQ ID NO: 197 - DNA, 20 bp, synthetic construct
  source 1..20: mol_type = other DNA
gccggaagacactatgaagc

SEQ ID NO: 198 - DNA, 377 bp, synthetic construct
  source 1..377: mol_type = other DNA
ttgtttatggatgcgctggggttgtcgatggcgctcggtacgtttattgcgggtgtgctactggcggaaagtgaatatcgccatgaactggaaacggctatcgatcccttcaaaggcttgctgctcggtttgttctttatctctgtcggcatgtcgctcaacctcggggtgctttatacccatctgttgtgggtagtgataagtgtggttgtgctggtggcggtgaaaattctcgtgctgtatctgctggcgcgattgtatggcgtgcgcagttctgagcggatgcagtttgctggcgtgttgagtcagggcggtgagtttgcctttgtcctcttttctaccgcttcttcacaacgcttattccagggcgaccagat

SEQ ID NO: 199 - DNA, 331 bp, synthetic construct
  source 1..331: mol_type = other DNA
ttgcatattcttgcgcgagcgcgcggacgtgtggaagcgcatgagttattacaggcaggggtgacgcagttttcccgtgaaacattctccagtgcgttagagctggggcgcaagacgctggtcacgcttggcatgcatccgcatcaggcgcagcgcgcgcaactgcattttcgccgcctggatatgcgaatgctgcgggagttaatcccgatgcatgctgataccgtacaaatttctcgcgccagggaagcccgacgtgaactggaagagattttccagcgtgaaatgcaacaagaacgacgccagctggacggctgggatgaatttgagt

SEQ ID NO: 200 - DNA, 20 bp, synthetic construct
  source 1..20: mol_type = other DNA
ggcgagttaacgacgacaca

SEQ ID NO: 201 - DNA, 432 bp, synthetic construct
  source 1..432: mol_type = other DNA
gcgctaaaagctattgaagcggagccgcgcacgctgattttttatgaatctacccaccgtctgttagatagcctggaagatatcgttgcggtattaggcgaatcccgttacgtggttctggcgcgtgagctaaccaaaacctgggaaaccattcacggcgcgcccgttggcgagctgctggcgtgggtaaaagaagatgaaaaccgtcgcaaaggcgaaatggtgctgattgtcgaaggccataaagcgcaggaaaatgacttgcctgctgatgccctgcgcacgctggcgctgctacaggcagaactgccgctgaaaaaagcggcggcgctggccgcagaaattcacggcgtgaagaaaaatgcgctgtataagtatgcgctggagcagcagggagagtgattacaggcgtcgcagcaggaatagcgctac

SEQ ID NO: 202 - DNA, 455 bp, synthetic construct
  source 1..455: mol_type = other DNA
tcacgcatgtgaaatggttatgcagccataaaaatgaagccgggatagcggtggagactttagccgtgagaaaacgttctgtcgcatcctgttttccttcgccagtcaccagtaacaaaacttcgcgggcattgagaatatccttcaggcctaaggtgatcccacgagtcacgggacggtccgcggtttttaacatctcatgttgctgtgttctggcatcaagttgactgatatggcaggctggttgcaggctttctcccggttcgttcagcccaagatgaccgtttttccccaatccgagaacgcataaatccagaccgcctttgcgcgcaatcaggttcgttacccgttcgcactctgtctcatttatctcttcggagcgaaagctgatgagctggtcttcacgcagccccagcggctgcacgatatgctgttgtaggaaagtttcgcaggtg

SEQ ID NO: 203 - DNA, 20 bp, synthetic construct
  source 1..20: mol_type = other DNA
ttgcgtattttcaaaaagcg

SEQ ID NO: 204 - DNA, 477 bp, synthetic construct
  source 1..477: mol_type = other DNA
accagccgagattcaacaggttgttgcccgtcaggcgaccaatcaaaaactccattgagatgtagttaacatgtcgctgattcgccactggcttggcgaatggctgagcacgcagcatttcggccagtgcttcgctcactgccagccaccactggcgaggagtcatttcagccgcagaatttaagccataacgctgccactgacgtgaaagcgcttcctgaaattgcttatcgttaaaaataggttgtgacataggagttccacttttcttagattttcaacacaacgttatcgctagtttgccaggctcgatgttgaccttcctcatcctgcgggggattaggcagggaggagttgcggggatgagcaaggaaatgtgatctcgaccacttaaagctagtgcaatccacaggattagcagcaaatcaatgccataccgcgcagaaaatctgtatctaagtgcaaaaaatggccgtt

SEQ ID NO: 205 - DNA, 456 bp, synthetic construct
  source 1..456: mol_type = other DNA
cgtattttcaaaaagcggaaggtaactctataaattaagtaaaggagtgaaacagtttcacaagtaaaatatcaagtgtgctccatctcattcttaatagatttattaagatcatctttttagatggcactttcatcagaaatgaagaagaaacccttgcttaaatgaaactgatgaacataaggaaaataccgtacaacccagtattcacgctggatcagcgtcgttttaggtgagttgttaataaacatttggaattgtgacacagtgcaaattcagacacataaaaaaacgtcatcgcttgcattagaaaggtttctggccgaccttataaccattaattacgaagcgcaaaaaaaataatatttcctcattttccacagtgaagtgattaactatgctgattccgtcaaaattaagtcgtccggttcgactcgaccataccgtggttcgtga

SEQ ID NO: 206 - DNA, 20 bp, synthetic construct
  source 1..20: mol_type = other DNA
ccgtgacgttatccgcacca

SEQ ID NO: 207 - DNA, 357 bp, synthetic construct
  source 1..357: mol_type = other DNA
acgatgacctgatgcgtccggacttcaacaacgatgactacgctattgcttgctgcgtaagcccgatgatcgttggtaaacaaatgcagttcttcggtgcgcgtgcaaacctggcgaaaaccatgctgtacgcaatcaacggcggcgttgacgaaaaactgaaaatgcaggttggtccgaagtctgaaccgatcaaaggcgatgtcctgaactatgatgaagtgatggagcgcatggatcacttcatggactggctggctaaacagtacatcactgcactgaacatcatccactacatgcacgacaagtacagctacgaagcctctctgatggcgctgcacgaccgtgacgttatcc

SEQ ID NO: 208 - DNA, 442 bp, synthetic construct
  source 1..442: mol_type = other DNA
gtgacgctatcccgactcagtctgttctgaccatcacttctaacgttgtgtatggtaagaaaactggtaacaccccagacggtcgtcgtgctggcgcgccgttcggaccgggtgctaacccgatgcacggtcgtgaccagaaaggtgctgtagcgtctctgacttccgttgctaaactgccgtttgcttacgctaaagatggtatctcctacaccttctctatcgttccgaacgcactgggtaaagacgacgaagttcgtaagaccaacctggctggtctgatggatggttacttccaccacgaagcatccatcgaaggtggtcagcacctgaacgttaacgtgatgaaccgtgaaatgctgctcgacgcgatggaaaacccggaaaaatatccgcagctgaccatccgtgtatctggctacgcagtacgtttcaactcgct

SEQ ID NO: 209 - DNA, 20 bp, synthetic construct
  source 1..20: mol_type = other DNA
gttatcgtgatgcgcattct

SEQ ID NO: 210 - DNA, 458 bp, synthetic construct
  source 1..458: mol_type = other DNA
tttccgcagccagcgattatcgcgccgcagcgcaacgcattctgccgccgttcctgttccactatatggatgggggggcatattctgaatacacgctgcgccgcaacgtggaagatttgtcagaagtggcgctgcgccagcgtattctgaaaaacatgtctgacttaagcctggaaacgacgctgtttaatgagaaattgtcgatgccggtggcgctaggtccggtaggtttgtgtggcatgtatgcgcgacgcggcgaagttcaggctgccaaagcagcagatgcgcatggcattccgtttactctctcgacggtttccgtttgcccgattgaagaagtggctccggctatcaaacgtccgatgtggttccagctttatgtgctgcgcgatcgcggctttatgcgtaacgccctggagcgagcaaaagccgcgggttgttcgacgctggttttcacc

SEQ ID NO: 211 - DNA, 442 bp, synthetic construct
  source 1..442: mol_type = other DNA
gatccgcgatttctgggatggcccgatggtgatcaaagggatcctcgatccggaagatgcgcgcgatgcagtacgttttggtgctgatggaattgtggtttctaaccacggtggccgccagttagatggcgtactctcttctgctcgtgcactgcctgctattgcggatgcggtgaaaggtgatatcgccattctggcggatagcggaatacgtaacgggcttgatgtcgtgcgtatgattgcgctcggtgccgacaccgtactgctgggtcgtgctttcctgtatgcactggcaacagcgggccaggcgggtgtagctaatctgctaaatctgatcgaaaaagagatgaaagtggcgatgacgctgactggcgcgaaatcgattagcgaaattacgcaagattcgctggtgcaggggctgggtaaagagttgcctgcggca

SEQ ID NO: 212 - DNA, 20 bp, synthetic construct
  source 1..20: mol_type = other DNA
taacacccagcccgatgccc

SEQ ID NO: 213 - DNA, 357 bp, synthetic construct
  source 1..357: mol_type = other DNA
ttctgcatagcaggtgaggcaaatgagatttattcgccactacccagtatggatgagatctgaaaaagggagaggaaaattgcccggtagccttcactaccgggcgcaggcttagatggaggtacggcggtagtcgcggtattcggcgtgccagaaattatcatcaatggcctgttgcagagcttcggcagacgttttcaccgccacgccttgctgctgcgccattttgccaaccgcaaaggcaattgcgcgggagactttctgaatatctttcagttccggcagtaccagaccttcgccgttcaggaccagcggcgaatactgagcaagcatttcacttgccgacatcagcatctc

SEQ ID NO: 214 - DNA, 574 bp, synthetic construct
  source 1..574: mol_type = other DNA
gagattttcgcgcttctgcaccagtttggtctggaaaggcagcaggttcggcatcttgtcggtcagcaggccaaagcgatcgaccataaagactttctgccgcgccgcttcctcgcttaatccttcgcgctgggtctgggcgatgatcatttcggcaatgccgcatcccgctgaacctgcgccaaggaagacgatttttttctcgcttaactgaccacctgccgcgcggctggctgcgatcagtgtgccgactgttaccgccgcggtgccctgaatgtcatcgttaaaagaacaaatttcattgcgatagcggttaagtaacggcatcgcatttttttgtgcgaagtcttcaaactgcaacagtacgtccggccagcgttgtttcacagcctggataaattcatcaacaaattcatagtattcgtcgtcagtgatacgcggattacgccagcccatatacagcggatcgttaagcagctgttggttgttggtgccgacatccagcaccaccggaagggtataggccggactgatgccgccacaggcggtatagagcgacagtttaccgatcgga

SEQ ID NO: 215 - DNA, 8553 bp, synthetic construct
  source 1..8553: mol_type = other DNA
gaattccggatgagcattcatcaggcgggcaagaatgtgaataaaggccggataaaacttgtgcttatttttctttacggtctttaaaaaggccgtaatatccagctgaacggtctggttataggtacattgagcaactgactgaaatgcctcaaaatgttctttacgatgccattgggatatatcaacggtggtatatccagtgatttttttctccattttagcttccttagctcctgaaaatctcgataactcaaaaaatacgcccggtagtgatcttatttcattatggtgaaagttggaacctcttacgtgccgatcaacgtctcattttcgccaaaagttggcccagggcttcccggtatcaacagggacaccaggatttatttattctgcgaagtgatcttccgtcacaggtatttattcgtccgagacataaggcgcatccggtaatttatccagttgctggcgcagcataaaaatcagctcaaatacatgatcgggcagcgtaatttcaccaatctctttctgccagcgttcatattcttcatctgtgatctgcaaggaggcaggaaccggattgtcattttcatcctgttgactggtcagcatggagcggaaattcgctttatcctgcactttatctaaccacagacgaatcagcatgcgatcatataacgcttccagactgctgtctgcttccggcagctcgttggaggccgccaccagcagacgcatcgggattttttctacgagtgcgccgttgcggaactggcgctcgttaatggcggtgagcagggtattaagaattgccggacccgctttccagatctcatccagaaagacgatttcagcttccggcaggtaaccgctggttaaacgttcatagcgcccttcatcttttagcgcctgaatagaaaggggaccaaaaacttcttccggcgtggagaagcgggtcatcagatattcaaacgcgcgggtctagagcttgtcgacgtctcgagtttatggctagctcagtcctaggtacaatgctagcctcgaggaaagaggagaaagaagcttatgaatattcgtccattgcatgatcgcgtgatcgtcaagcgtaaagaagttgaaactaaatctgctggcggcatcgttctgaccggctctgcagcggctaaatccacccgcggcgaagtgctggctgtcggcaatggccgtatccttgaaaatggcgaagtgaagccgctggatgtgaaagttggcgacatcgttattttcaacgatggctacggtgtgaaatctgagaagatcgacaatgaagaagtgttgatcatgtccgaaagcgacattctggcaattgttgaagcgtaatccgcgcacgacactgaacatacgaatttaaggaataaagataatggcagctaaagacgtaaaattcggtaacgacgctcgtgtgaaaatgctgcgcggcgtaaacgtactggcagatgcagtgaaagttaccctcggtccaaaaggccgtaacgtagttctggataaatctttcggtgcaccgaccatcaccaaagatggtgtttccgttgctcgtgaaatcgaactggaagacaagttcgaaaatatgggtgcgcagatggtgaaagaagttgcctctaaagcaaacgacgctgcaggcgacggtaccaccactgcaaccgtactggctcaggctatcatcactgaaggtctgaaagctgttgctgcgggcatgaacccgatggacctgaaacgtggtatcgacaaagcggttaccgctgcagttgaagaactgaaagcgctgtccgtaccatgctctgactctaaagcgattgctcaggttggtaccatctccgctaactccgacgaaaccgtaggtaaactgatcgctgaagcgatggacaaagtcggtaaagaaggcgttatcaccgttgaagacggtaccggtctgcaggacgaactggacgtggttgaaggtatgcagttcgaccgtggctacctgtctccttacttcatcaacaagccggaaactggcgcagtagaactggaaagcccgttcatcctgctggctgacaagaaaatctccaacatccgcgaaatgctgccggttctggaagctgttgccaaagcaggcaaaccgctgctgatcatcgctgaagatgtagaaggcgaagcgctggcaactctggttgttaacaccatgcgtggcatcgtgaaagtcgctgcggttaaagcaccgggcttcggcgatcgtcgtaaagctatgctgcaggatatcgcaaccctgactggcggtaccgtgatctctgaagagatcggtatggagctggaaaaagcaaccctggaagacctgggtcaggctaaacgtgttgtgatcaacaaagacaccaccactatcatcgatggcgtgggtgaagaagctgcaatccagggccgtgttgctcagatccgtcagcagattgaagaagcaacttctgactacgaccgtgaaaaactgcaggaacgcgtagcgaaactggcaggcggcgttgcagttatcaaagtgggtgctgctaccgaagttgaaatgaaagagaaaaaagcacgcgttgaagatgccctgcacgcgacccgtgctgcggtagaagaaggcgtggttgctggtggtggtgttgcgctgatccgcgtagcgtctaaactggctgacctgcgtggtcagaacgaagaccagaacgtgggtatcaaagttgcactgcgtgcaatggaagctccgctgcgtcagatcgtattgaactgcggcgaagaaccgtctgttgttgctaacaccgttaaaggcggcgacggcaactacggttacaacgcagcaaccgaagaatacggcaacatgatcgacatgggtatcctggatccaaccaaagtaactcgttctgctctgcagtacgcagcttctgtggctggcctgatgatcaccaccgaatgcatggttaccgacctgccgaaaaacgatgcagctgacttaggcgctgctggcggtatgggcggcatgggtggcatgggcggcatgatgtaattgccctgcacctcgcagaaataaacaaacccccctgtgattttttgaggtaacaagatgcaagtttcagttgaaaccactcaaggccttggccgccgtgtaacgattactatcgctgctgacagcatcgagaccgctgttaaaagcgagctggtcaacgttgcgaaaaaagtacgtattgacggcttccgcaaaggcaaagtgccaatgaatatcgttgctcagcgttatggcgcgtctgtacgccaggacgttctgggtgacctgatgagccgtaacttcattgacgccatcattaaagaaaaaatcaatccggctggcgcaccgacttatgttccgggcgaatacaagctgggtgaagacttcacttactctgtagagtttgaagtttatccggaagttgaactgcagggtctggaagcgatcgaagttgaaaaaccgatcgttgaagtgaccgacgctgacgttgacggcatgctggatactctgcgtaaacagcaggcgacctggaaagaaaaagacggcgctgttgaagcagaagaccgcgtaaccatcgacttcaccggttctgtagacggcgaagagttcgaaggcggtaaagcgtctgatttcgtactggcgatgggccagggtcgtatgatcccgggctttgaagacggtatcaaaggccacaaagctggcgaagagttcaccatcgacgtgaccttcccggaagaataccacgcagaaaacctgaaaggtaaagcagcgaaattcgctatcaacctgaagaaagttgaagagcgtgaactgccggaactgactgcagaattcatcaaacgtttcggcgttgaagatggttccgtagaaggtctgcgcgctgaagtgcgtaaaaacatggagcgcgagctgaagagcgccatccgtaaccgcgttaagtctcaggcgatcgaaggtctggtaaaagctaacgacatcgacgtaccggctgcgctgatcgacagcgaaatcgacgttctgcgtcgccaggctgcacagcgtttcggtggcaacgaaaaacaagctctggaactgccgcgcgaactgttcgaagaacaggctaaacgccgcgtagttgttggcctgctgctgggcgaagttatccgcaccaacgagctgaaagctgacgaagagcgcgtgaaaggcctgatcgaagagatggcttctgcgtacgaagatccgaaagaagttatcgagttctacagcaaaaacaaagaactgatggacaacatgcgcaatgttgctctggaagaacaggctgttgaagctgtactggcgaaagcgaaagtgactgaaaaagaaaccactttcaacgagctgatgaaccagcaggcgtaatgagatgccccgatcctggagatatggatgaaatcactgtttaaagtaacgctgctggcgaccacaatggccgttgccctgcatgcaccaatcacttttgctgctgaagctgcaaaacctgctacaactgctgacagcaaagcagcgttcaaaaatgacgatcagaaatcagcttatgcactgggtgcttcgctgggtcgttacatggaaaactctcttaaagaacaagaaaaactgggcatcaaactggataaagatcagctgatcgctggtgttcaggatgcatttgctgataagagcaaactttccgaccaagagatcgaacagactctgcaagcattcgaagctcgcgtgaagtcttctgctcaggcgaagatggaaaaagacgcggctgataacgaagcaaaaggtaaagagtaccgcgagaaatttgccaaagagaaaggtgtgaaaacctcttccactggtctggtttatcaggtagtagaagccggtaaaggcgaagccccgaaagacagcgatactgttgtagtgaactacaaaggtacgctgatcgacggtaaagagttcgacaactcttacacccgtggtgaaccgctctctttccgtctggacggtgttatcccgggttggacagaaggtctgaagaacatcaagaaaggcggtaagatcaaactggttattccaccagaactggcttacggcaaagcgggtgttccggggatcccaccgaattctaccctggtgtttgacgtagagctgctggatgtgaaaccagcgccgaaggctgatgcaaagccggaagctgatgcgaaagccgcagattctgctaaaaaataattgaaatggaaaaagtatgaagaactggaaaacgctgcttctcggtatcgccatgatcgcgaataccagtttcgctgccccccaggtagtcgataaagtcgcagccgtcgtcaataacggcgtcgtgctggaaagcgacgttgatggattaatgcagtcggtaaaactgaacgctgctcaggcaaggcaacaacttcctgatgacgcgacgctgcgccaccaaatcatggagcgtttgatcatggatcaaatcatcctgcagatggggcagaaaatgggagtgaaaatctccgatgagcagctggatcaggcgattgctaacatcgcgaaacagaacaacatgacgctggatcagatgcgcagccgtctggcttacgatggtctgaactacaacacctatcgtaaccagatccgcaaagagatgattatctctgaagtgcgtaacaacgaggtgcgtcgtcgcatcaccatcctgccgcaggaagtcgaatccctggcgcagcaagtgggtaaccaaaacgacgccagcactgagctgaacctgagccacatcctgatcccactgccggaaaacccgacctctgatcaggtgaacgaagcggaaagccaggcgcgcgcgattgtcgatcaggcgcgtaacggcgctgatttcggtaagctggcgattgctcattctgccgaccagcaggcgctgaacggcggacagatgggctggggccgtattcaggagttgccggggatcttcgcccaggcattaagcaccgcgaagaaaggcgacattgttggcccgattcgttccggcgttggcttccatattctgaaagttaacgacctgcgcggcgaaagcaaaaatatctcggtgaccgaagttcatgctcgccatattctgctgaaaccgtcgccgatcatgactgacgaacaggcccgcgtgaaactggaacagattgctgccgatatcaagagtggtaaaacgacttttgctgccgcagcgaaagagttctctcaggatccaggctctgctaaccagggcggtgatctcggctgggctacaccagatattttcgatccggccttccgtgacgccctgacccgcctgaacaaaggtcaaatgagtgcaccggttcactcttcattcggctggcatttaatcgaactgctggatacccgtaatgtcgataaaaccgacgcggcacagaaagatcgtgcataccgcatgctgatgaaccgtaagttctcggaagaagcagcaagctggatgcaggaacaacgtgccagcgcctacgttaaaatcctgagcaactaataacgagctcgatagtgctagtgtagatcgctactagagccaggcatcaaataaaacgaaaggctcagtcgaaagactgggcctttcgttttatctgttgtttgtcggtgaacgctctctactagagtcacactggctcaccttcgggtgggcctttctgcgtttatatactagaagcggccgaatgtggccgcatttaggagtacgattttgccgttaatcgtgcatactgtgcgcttttttgtgggccaagggactaagcacacatttcatatttcaacgaaagactagtctatgagcactgataataagcaatcattgcccgcgattaccctcgcggcgattggagttgtctacggcgatattggtaccagcccgttatatacacttcgtgaatgtttgtccggccagtttggttttggcgttgaacgcgatgccgtgtttggctttttatcgctgatcttctggctgctaatctttgtggtttccattaaatatctcaccttcgtgatgcgggcagatatgcaggaattcaaaaaaagcaccgactcggtgccactttttcaagttgataacggactagccttattttaacttgctatttctagctctaaaaccttcattatggctcaccctcactagtattatacctaggactgagctagctgtcaaggatccagcatcgctcactgactcgctacgctcggtcgttcgactgcggcgagcggaaatggcttacgaacggggcggagatttcctggaagatgccaggaagatacttaacagggaagtgagagggccgcggcaaagccgtttttccataggctccgcccccctgacaagcatcacgaaatctgacgctcaaatcagtggtggcgaaacccgacaggactataaagataccaggcgtttccccctggcggctccctcgtgcgctctcctgttcctgcctttcggtttaccggtgtcattccgctgttatggccgcgtttgtctcattccacgcctgacactcagttccgggtaggcagttcgctccaagctggactgtatgcacgaaccccccgttcagtccgaccgctgcgccttatccggtaactatcgtcttgagtccaacccggaaagacatgcaaaagcaccactggcagcagccactggtaattgatttagaggagttagtcttgaagtcatgcgccggttaaggctaaactgaaaggacaagttttggtgactgcgctcctccaagccagttacctcggttcaaagagttggtagctcagagaaccttcgaaaaaccgccctgcaaggcggttttttcgttttcagagcaagagattacgcgcagaccaaaacgatctcaagaagatcatctgtaggtcgttcgctccaagctggaaggatcttcacctagatccttttaaattaaaaatgaagttttaaatcaatctaaagtatatatgagtaaacttggtctgacagaatttctgccattcatccgcttattatcacttattcaggcgtagcaaccaggcgtttaagggcaccaataactgccttaaaaaaattacgccccgccctgccactcatcgcagtactgttgtaattcattaagcattctgccgacatggaagccatcacaaacggcatgatgaacctgaatcgccagcggcatcagcaccttgtcgccttgcgtataatatttgcccatggtgaaaacgggggcgaagaagttgtccatattggccacgtttaaatcaaaactggtgaaactcacccagggattggctgagacgaaaaacatattctcaataaaccctttagggaaataggccaggttttcaccgtaacacgccacatcttgcgaatatatgtgtagaaactgccggaaatcgtcgtggtattcactccagagcgatgaaaacgtttcagtttgctcatggaaaacggtgtaacaagggtgaacactatcccatatcaccagctcaccgtctttcattgccatacg

SEQ ID NO: 216 - DNA, 8235 bp, synthetic construct
  source 1..8235: mol_type = other DNA
gaattccggatgagcattcatcaggcgggcaagaatgtgaataaaggccggataaaacttgtgcttatttttctttacggtctttaaaaaggccgtaatatccagctgaacggtctggttataggtacattgagcaactgactgaaatgcctcaaaatgttctttacgatgccattgggatatatcaacggtggtatatccagtgatttttttctccattttagcttccttagctcctgaaaatctcgataactcaaaaaatacgcccggtagtgatcttatttcattatggtgaaagttggaacctcttacgtgccgatcaacgtctcattttcgccaaaagttggcccagggcttcccggtatcaacagggacaccaggatttatttattctgcgaagtgatcttccgtcacaggtatttattcgaacgaaacgctatcgataagaataaaaaggaataaaagtggaatataaagtctggcacttcttactgaccacgcaaacacctttcgtacagcatgatgagagcggcaaaagcaaactacacttatgcttcattcgatgcacatttgcagaaggttgccgctatgaagccaacgatgctactcatgattaccgtattcctgatttttccagccatttctcaggccgagtcgccattcagttctctacagtcggcaaaagagaaaaccacggtattgcaagatttacgtaaaatttgcacgccacaggcgtcattatcagatgaagcgtgggaaaagttaatgttgtcagatgaaaacaataaacaacatatacgcgaggccatcgtggcgatggaacgtaataatcagagcaattattgggaagcgttgggtaaggtagaatgcccggatatgtaagaacggcaacaaccactgtctagagcttgtcgacgtctcgagtttatggctagctcagtcctaggtacaatgctagcctcgaggaaagaggagaaagaagcttatgaaaaagatttggctggcgctggctggtttagttttagcgtttagcgcatcggcggcgcagtatgaagatggtaaacagtacactaccctggaaaaaccagttgctggcgcgccgcaagtgctggagtttttctctttcttctgcccgcactgctatcagtttgaagaagttctgcatatttctgataacgtgaagaaaaaactgccggaaggcgtgaagatgactaaataccacgtcaacttcatggggggtgacctgggcaaagagctgactcaggcatgggctgtggcgatggcgctgggcgtggaagacaaagtcacagttccgctgtttgaaggcgtacaaaaaacccagaccattcgttcagcatctgatatccgcgatgtatttatcaacgcaggtattaaaggtgaagagtacgacgcggcgtggaacagcttcgtggtgaaatctctggtcgctcagcaggaaaaagctgcagctgacgtgcaattgcgtggtgttccggcgatgtttgttaacggtaaatatcagctgaatccgcagggtatggataccagcaatatggatgtttttgttcagcagtatgctgatacagtgaaatatctgtccgagaaaaaataacgagggcaaaaaatgaagaaaggttttatgttgtttactttgttggcagcgttttcaggctttgttcaggctgatgacgcggcaattcaacaaacgttagccaaaatgggcatcaaaagcagcgatattcagcccgcgcccgtagctggcatgaagacagttctgactaacagcggtgtgttgtacatcaccgatgatggtaaacatatcattcaggggccaatgtatgacgttagtggcacggctccggtcaatgtcaccaataagatgctgttaaagcagttgaatgcgcttgaaaaagagatgatcgtttataaagcgccgcaggaaaaacacgtcatcaccgtgtttactgatattacctgtggttactgccacaaactgcatgagcaaatggcagactataacgcgctggggatcaccgtgcgttatcttgctttcccgcgccaggggctggacagcgatgcagagaaagaaatgaaagctatctggtgtgcgaaagataaaaacaaagcgtttgatgatgtgatggcaggtaaaagcgtcgcaccagccagctgcgacgtggatattgccgaccattacgcacttggcgtccagcttggcgttagcggtactccggcagttgtgctgagcaatggcacacttgttccgggttaccagccgccgaaagacatgaaagaattcctcgacgaacaccaaaaaatgaccagcggtaaataaggctatggattgtggagacgtttagatgggtaaaataattggtatcgacctgggtactaccaactcttgtgtagcgattatggatggcaccactcctcgcgtgctggagaacgccgaaggcgatcgcaccacgccttctatcattgcctatacccaggatggtgaaactctagttggtcagccggctaaacgtcaggcagtgacgaacccgcaaaacactctgtttgcgattaaacgcctgattggtcgccgcttccaggacgaagaagtacagcgtgatgtttccatcatgccgttcaaaattattgctgctgataacggcgacgcatgggtcgaagttaaaggccagaaaatggcaccgccgcagatttctgctgaagtgctgaaaaaaatgaagaaaaccgctgaagattacctgggtgaaccggtaactgaagctgttatcaccgtaccggcatactttaacgatgctcagcgtcaggcaaccaaagacgcaggccgtatcgctggtctggaagtaaaacgtatcatcaacgaaccgaccgcagctgcgctggcttacggtctggacaaaggcactggcaaccgtactatcgcggtttatgacctgggtggtggtactttcgatatttctattatcgaaatcgacgaagttgacggcgaaaaaaccttcgaagttctggcaaccaacggtgatacccacctggggggtgaagacttcgacagccgtctgatcaactatctggttgaagaattcaagaaagatcagggcattgacctgcgcaacgatccgctggcaatgcagcgcctgaaagaagcggcagaaaaagcgaaaatcgaactgtcttccgctcagcagaccgacgttaacctgccatacatcactgcagacgcgaccggtccgaaacacatgaacatcaaagtgactcgtgcgaaactggaaagcctggttgaagatctggtaaaccgttccattgagccgctgaaagttgcactgcaggacgctggcctgtccgtatctgatatcgacgacgttatcctcgttggtggtcagactcgtatgccaatggttcagaagaaagttgctgagttctttggtaaagagccgcgtaaagacgttaacccggacgaagctgtagcaatcggtgctgctgttcagggtggtgttctgactggtgacgtaaaagacgtactgctgctggacgttaccccgctgtctctgggtatcgaaaccatgggcggtgtgatgacgacgctgatcgcgaaaaacaccactatcccgaccaagcacagccaggtgttctctaccgctgaagacaaccagtctgcggtaaccatccatgtgctgcagggtgaacgtaaacgtgcggctgataacaaatctctgggtcagttcaacctagatggtatcaacccggcaccgcgcggcatgccgcagatcgaagttaccttcgatatcgatgctgacggtatcctgcacgtttccgcgaaagataaaaacagcggtaaagagcagaagatcaccatcaaggcttcttctggtctgaacgaagatgaaatccagaaaatggtacgcgacgcagaagctaacgccgaagctgaccgtaagtttgaagagctggtacagactcgcaaccagggcgaccatctgctgcacagcacccgtaagcaggttgaagaagcaggcgacaaactgccggctgacgacaaaactgctatcgagtctgcgctgactgcactggaaactgctctgaaaggtgaagacaaagccgctatcgaagcgaaaatgcaggaactggcacaggtttcccagaaactgatggaaatcgcccagcagcaacatgcccagcagcagactgccggtgctgatgcttctgcaaacaacgcgaaagatgacgatgttgtcgacgctgaatttgaagaagtcaaagacaaaaaataatcgccctataaacgggtaattatactgacacgggcgaaggggaatttcctccccgcccgtgcattcatctaggggcaatttaaaaaagatggctaagcaagattattacgagattttaggcgtttccaaaacagcggaagagcgtgaaatcagaaaggcctacaaacgcctggccatgaaataccacccggaccgtaaccagggtgacaaagaggccgaggcgaaatttaaagagatcaaggaagcttatgaagttctgaccgactcgcaaaaacgtgcggcatacgatcagtatggtcatgctgcgtttgagcaaggtggcatgggcggcggcggttctggcggcggcgcagacttcagcgatatttttggtgacgttttcggcgatatttttggcggcggacgtggtcgtcaacgtgcggcgcgcggtgctgatttacgctataacatggagctcaccctcgaagaagctgtacgtggcgtgaccaaagagatccgcattccgactctggaagagtgtgacgtttgccacggtagcggtgcaaaaccaggtacacagccgcagacttgtccgacctgtcatggttctggtcaggtgcagatgcgccagggattcttcgctgtacagcagacctgtccacactgtcagggccgcggtacgctgatcaaagatccgtgcaacaaatgtcatggtcatggtcgtgttgagcgcagcaaaacgctgtccgttaaaatcccggcaggggtggacactggagaccgcatccgtcttgcgggcgaaggtgaagcgggcgagcatggcgcaccggcaggcgatctgtacgttcaggttcaggttaaacagcacccgattttcgagcgtgaaggcaacaacctgtattgcgaagtcccgatcaacttcgctatggcggcgctgggtggcgaaatcgaagtaccgacccttgatggtcgcgtcaaactgaaagtgcctggcgaaacccagaccggtaagctattccgtatgcgcggtaaaggcgtcaagtctgtccgcggtggcgcgcagggtgatttgctgtgccgcgttgtcgtcgaaacaccggtaggcctgaacgaaaggcagaaacagctgctgcaagagctgcaagaaagcttcggtggcccaaccggcgagcacaacagcccgcgctcaaagagcttctttgatggtgtgaagaagttttttgacgacctgacccgctaacctcgcggagaaattcatgagtagtaaagaacagaaaacgcctgaggggcaagccccggaagaaattatcatggatcagcacgaagagattgaggcagttgagccagaagcttctgctgagcaggtggatccgcgcgatgaaaaagttgcgaatctcgaagctcagctggctgaagcccagacccgtgaacgtgacggcattttgcgtgtaaaagccgaaatggaaaacctgcgtcgtcgtactgaactggatattgaaaaagcccacaaattcgcgctggagaaattcatcaacgaattgctgccggtgattgatagcctggatcgtgcgctggaagtggctgataaagctaacccggatatgtctgcgatggttgaaggcattgagctgacgctgaagtcgatgctggatgttgtgcgtaagtttggcgttgaagtgatcgccgaaactaacgtcccactggacccgaatgtgcatcaggccatcgcaatggtggaatctgatgacgttgcgccaggtaacgtactgggcattatgcagaagggttatacgctgaatggtcgtacgattcgtgcggcgatggttactgtagcgaaagcaaaagcttaataacgagctcgatagtgctagtgtagatcgctactagagccaggcatcaaataaaacgaaaggctcagtcgaaagactgggcctttcgttttatctgttgtttgtcggtgaacgctctctactagagtcacactggctcaccttcgggtgggcctttctgcgtttatatactagaagcggccgaccaacgcttctttacctgatatcaggatttcttcattttcacctttgcagtcaccaacaatgcagtcagcaacatcaatgtgccggacaacatcagcggcgaagtcagaccaatgttatccaacgcataaccgccgattgccgcaccgcaggtgttagcaagctgaataacggccacctgaatagatccagccttttctgcctgatcggccaatgagcgagtgatccacgttgaccaaccaacgggaattaaagcaaaggtcagcccccagataatcgcaacaccagtagcaacaattttatagcttccccacagcgtcagtaccagcgcgctcagggcgagcacaaacggtgcgcccgctaaggccagtttcaccgaacgtttgagaataaacgacgaaagcgatgtcccgacaaagctggcgataccaaaactcagcagcaccagggttaagccatcaacatgcaggaattcaaaaaaagcaccgactcggtgccactttttcaagttgataacggactagccttattttaacttgctatttctagctctaaaacctgaccaacgcttctttaccactagtattatacctaggactgagctagctgtcaaggatccagcatcgctcactgactcgctacgctcggtcgttcgactgcggcgagcggaaatggcttacgaacggggcggagatttcctggaagatgccaggaagatacttaacagggaagtgagagggccgcggcaaagccgtttttccataggctccgcccccctgacaagcatcacgaaatctgacgctcaaatcagtggtggcgaaacccgacaggactataaagataccaggcgtttccccctggcggctccctcgtgcgctctcctgttcctgcctttcggtttaccggtgtcattccgctgttatggccgcgtttgtctcattccacgcctgacactcagttccgggtaggcagttcgctccaagctggactgtatgcacgaaccccccgttcagtccgaccgctgcgccttatccggtaactatcgtcttgagtccaacccggaaagacatgcaaaagcaccactggcagcagccactggtaattgatttagaggagttagtcttgaagtcatgcgccggttaaggctaaactgaaaggacaagttttggtgactgcgctcctccaagccagttacctcggttcaaagagttggtagctcagagaaccttcgaaaaaccgccctgcaaggcggttttttcgttttcagagcaagagattacgcgcagaccaaaacgatctcaagaagatcatctgtaggtcgttcgctccaagctggaaggatcttcacctagatccttttaaattaaaaatgaagttttaaatcaatctaaagtatatatgagtaaacttggtctgacagaatttctgccattcatccgcttattatcacttattcaggcgtagcaaccaggcgtttaagggcaccaataactgccttaaaaaaattacgccccgccctgccactcatcgcagtactgttgtaattcattaagcattctgccgacatggaagccatcacaaacggcatgatgaacctgaatcgccagcggcatcagcaccttgtcgccttgcgtataatatttgcccatggtgaaaacgggggcgaagaagttgtccatattggccacgtttaaatcaaaactggtgaaactcacccagggattggctgagacgaaaaacatattctcaataaaccctttagggaaataggccaggttttcaccgtaacacgccacatcttgcgaatatatgtgtagaaactgccggaaatcgtcgtggtattcactccagagcgatgaaaacgtttcagtttgctcatggaaaacggtgtaacaagggtgaacactatcccatatcaccagctcaccgtctttcattgccatacg

SEQ ID NO: 217 - DNA, 396 bp, synthetic construct
  source 1..396: mol_type = other DNA
ggtattacaatcccgcgtaatccgggttgtccgaatagtgaagataaaaattttccgcgtacagttatggttaatctgaatattcataaccgtaacacaaacaccaatccgaaacgtagtagcgattattataatcgtagcacaagcccgtggaatctgcatcgtaacgaagatccggaacgttatccaagcgttatctgggaagcaaaatgccgccatctgggttgtatcaatgcagatggtaacgttgattatcatatgaatagcgtgccgattcagcaggaaattctggttctgcgtcgtgaaccgccgcattgtccgaatagctttcgtctggaaaaaattctggttagcgttggttgtacctgtgttaccccgattgttcatcatgttgca

SEQ ID NO: 218 - protein, 132 aa, synthetic construct
GITIPRNPGCPNSEDKNFPRTVMVNLNIHNRNTNTNPKRSSDYYNRSTSPWNLHRNEDPERYPSVIWEAKCRHLGCINADGNVDYHMNSVPIQQEILVLRREPPHCPNSFRLEKILVSVGCTCVTPIVHHVA

SEQ ID NO: 219 - DNA, 459 bp, synthetic construct
  source 1..459: mol_type = other DNA
ctgcgtcgttgtctgattagcaccgatatgcatcatattgaagaaagctttcaggaaattaaacgtgccattcaggcaaaagatacctttccgaatgttaccattctgagcaccctggaaaccctgcagattatcaaaccactggatgtttgttgtgttaccaaaaatctgctggccttttatgttgatcgtgtttttaaagatcatcaggaaccgaatccgaaaattctgcgtaaaattagtagcattgccaatagctttctgtatatgcagaaaaccctgcgccagtgtcaggaacagcgtcagtgtcattgtcgtcaggaagcaaccaatgcaacccgtgtgattcatgataactatgatcagctggaagttcatgcagcagcgattaaaagcctgggtgaactggatgtgtttctggcatggattaataaaaatcatgaagtgatgtttagcgca

SEQ ID NO: 220 - protein, 153 aa, synthetic construct
LRRCLISTDMHHIEESFQEIKRAIQAKDTFPNVTILSTLETLQIIKPLDVCCVTKNLLAFYVDRVFKDHQEPNPKILRKISSIANSFLYMQKTLRQCQEQRQCHCRQEATNATRVIHDNYDQLEVHAAAIKSLGELDVFLAWINKNHEVMFSA

SEQ ID NO: 221 - DNA, 918 bp, synthetic construct
  source 1..918: mol_type = other DNA
atctgggaactgaaaaaggatgtttatgtggttgaactggattggtatccggatgcaccgggcgaaatggtggttctgacgtgtgatacgccggaagaagatggtattacctggacactggatcagagcagcgaagttctgggcagtggtaaaaccctgacgattcaggttaaagaatttggtgatgcaggtcagtatacctgtcataaaggtggtgaagttctgagccattccctgctgctgctgcataaaaaggaagatggtatctggagcaccgatattctgaaagatcagaaagaaccgaaaaacaaaacctttctgcgttgcgaagcgaaaaattattcaggccgttttacctgttggtggctgacgaccattagcacagatctgacctttagcgtgaaaagcagccgtggtagcagcgatccgcagggtgttacttgtggtgcagcaacgctgtctgcagaacgtgttcgtggtgataataaagaatatgaatatagcgtggaatgccaggaagattcagcatgtccggcagcagaagaaagcctgccgattgaagtgatggttgatgcagttcataaactgaaatatgaaaactataccagcagcttttttatccgtgatattattaaaccggaccctccgaaaaatctgcagctgaaacctctgaaaaatagtcgtcaggtggaagtgtcctgggaatatccggatacctggagcaccccacatagctattttagtctgaccttttgtgttcaggttcagggcaaatcaaaacgcgaaaaaaaagatcgtgtttttaccgataaaaccagcgcaaccgttatttgtcgtaaaaatgcaagcattagcgttcgtgcacaggatcgttattatagcagcagctggagcgaatgggcaagcgttccgtgtagc

SEQ ID NO: 222 - protein, 306 aa, synthetic construct
IWELKKDVYVVELDWYPDAPGEMVVLTCDTPEEDGITWTLDQSSEVLGSGKTLTIQVKEFGDAGQYTCHKGGEVLSHSLLLLHKKEDGIWSTDILKDQKEPKNKTFLRCEAKNYSGRFTCWWLTTISTDLTFSVKSSRGSSDPQGVTCGAATLSAERVRGDNKEYEYSVECQEDSACPAAEESLPIEVMVDAVHKLKYENYTSSFFIRDIIKPDPPKNLQLKPLKNSRQVEVSWEYPDTWSTPHSYFSLTFCVQVQGKSKREKKDRVFTDKTSATVICRKNASISVRAQDRYYSSSWSEWASVPCS

SEQ ID NO: 223 - DNA, 510 bp, synthetic construct
  source 1..510: mol_type = other DNA
cgtgcagttccgggtggtagcagcccggcatggacccagtgtcagcagctgagccagaaactgtgtaccctggcatggagcgcacatccgctggttggtcatatggatctgcgtgaagaaggtgatgaagaaaccaccaatgatgttccgcatattcagtgtggtgatggttgtgatccgcagggtctgcgtgataatagccagttttgtctgcagcgtattcatcagggtctgattttttatgaaaaactgctgggtagcgatatttttaccggtgaaccgagcctgctgccggatagcccggttggtcagctgcatgcaagcctgctgggtctgagccagctgctgcagccggaaggtcatcattgggaaacccagcagattccgagcctgagcccgagccagccgtggcagcgtctgctgctgcgttttaaaattctgcgtagcctgcaggcatttgttgcagttgcagcacgtgtttttgcacatggtgcagcaaccctgagcccg

SEQ ID NO: 224 - protein, 170 aa, synthetic construct
RAVPGGSSPAWTQCQQLSQKLCTLAWSAHPLVGHMDLREEGDEETTNDVPHIQCGDGCDPQGLRDNSQFCLQRIHQGLIFYEKLLGSDIFTGEPSLLPDSPVGQLHASLLGLSQLLQPEGHHWETQQIPSLSPSQPWQRLLLRFKILRSLQAFVAVAARVFAHGAATLSP

SEQ ID NO: 225 - DNA, 627 bp, synthetic construct
  source 1..627: mol_type = other DNA
cgcaaaggtccgccggcagcactgaccctgccgcgtgttcagtgtcgtgcatcccgctatccgattgcagttgattgtagttggaccctgccgccggcaccgaattccacctcaccggttagctttattgctacctatcgtctgggtatggccgcacgtggtcattcatggccttgtctgcagcagaccccgaccagcacgagctgtaccatcaccgatgttcagctgttttctatggcaccgtatgttctgaatgttacggcagttcatccgtggggttcaagcagctcttttgttccatttattaccgaacatatcatcaaaccggaccctccggaaggtgttcgtctgagcccgctggcagaacgtcagctgcaggttcagtgggaaccgccaggttcatggccgtttcctgaaatttttagcctgaaatattggattcgttataaacgtcagggtgcggcccgttttcatcgtgttggtcctattgaagcaacctcatttattctgcgtgcggtccgtcctcgtgcccgttattatgttcaggtcgccgcacaggatctgaccgattatggtgaactgagcgattggtcactgccggcaaccgcgaccatgtccctgggtaaa

SEQ ID NO: 226 - protein, 209 aa, synthetic construct
RKGPPAALTLPRVQCRASRYPIAVDCSWTLPPAPNSTSPVSFIATYRLGMAARGHSWPCLQQTPTSTSCTITDVQLFSMAPYVLNVTAVHPWGSSSSFVPFITEHIIKPDPPEGVRLSPLAERQLQVQWEPPGSWPFPEIFSLKYWIRYKRQGAARFHRVGPIEATSFILRAVRPRARYYVQVAAQDLTDYGELSDWSLPATATMSLGK

SEQ ID NO: 227 - DNA, 591 bp, synthetic construct
  source 1..591: mol_type = other DNA
cgtaacctgccggttgcgaccccggaccctggcatgtttccgtgtctgcatcattctcagaatctgctgcgtgcagtctctaatatgctgcagaaagcacgtcagaccctggaattttatccgtgtaccagtgaagaaatcgatcatgaagatattaccaaagataaaaccagcaccgtggaagcatgtctgccgctggaactgaccaaaaacgaaagctgtctgaacagccgcgaaaccagttttattacaaatggtagttgtctggcaagccgcaaaaccagctttatgatggcgctgtgtctgagctcaatttatgaagatctgaaaatgtatcaggtggaatttaaaaccatgaatgccaaactgctgatggaccctaaacgtcagatttttctggatcagaatatgctggcagttatcgatgaactgatgcaggcactgaactttaatagcgaaaccgttccgcagaaaagctccctggaagaaccggatttttataaaaccaaaatcaaactgtgcatcctgctgcatgcatttcgtattcgtgcagttaccattgatcgtgtgatgagctatctgaatgcaagc

SEQ ID NO: 228 - protein, 197 aa, synthetic construct
RNLPVATPDPGMFPCLHHSQNLLRAVSNMLQKARQTLEFYPCTSEEIDHEDITKDKTSTVEACLPLELTKNESCLNSRETSFITNGSCLASRKTSFMMALCLSSIYEDLKMYQVEFKTMNAKLLMDPKRQIFLDQNMLAVIDELMQALNFNSETVPQKSSLEEPDFYKTKIKLCILLHAFRIRAVTIDRVMSYLNAS

SEQ ID NO: 229 - DNA, 519 bp, synthetic construct
  source 1..519: mol_type = other DNA
gttcataccagtccgaaagtgaaaaatctgaatccgaaaaagtttagcatccatgatcaggatcataaagttctggtactggatagcggtaatctgattgcagtgccggataaaaattatattcgtccggaaattttttttgccctggcaagcagcctgagttcagcctcagcggaaaaaggtagcccgattctgctgggtgttagtaaaggtgaattttgtctgtattgtgataaagataaaggccagagccatccgagtctgcagctgaaaaaggaaaaactgatgaaactggcagcacagaaagaaagcgctcgtcgtccgtttattttttatcgtgcacaggtgggtagctggaatatgctggaaagcgcagcccatccaggttggtttatttgcaccagctgcaattgtaatgaaccggtgggtgttaccgataaatttgaaaatcgtaaacatatcgaatttagctttcagccggtttgtaaagcagaaatgagcccgagcgaagttagtgat

SEQ ID NO: 230 - protein, 173 aa, synthetic construct
VHTSPKVKNLNPKKFSIHDQDHKVLVLDSGNLIAVPDKNYIRPEIFFALASSLSSASAEKGSPILLGVSKGEFCLYCDKDKGQSHPSLQLKKEKLMKLAAQKESARRPFIFYRAQVGSWNMLESAAHPGWFICTSCNCNEPVGVTDKFENRKHIEFSFQPVCKAEMSPSEVSD

SEQ ID NO: 231 - DNA, 336 bp, synthetic construct
  source 1..336: mol_type = other DNA
gcactggataccaattattgtttttcaagcaccgaaaaaaattgttgtgttcgtcagctgtatattgattttcgtaaagatctgggttggaaatggattcatgaaccgaaaggttatcatgcaaatttttgtctgggtccgtgtccgtatatttggagcctggatacccagtatagcaaagttctggcactgtataatcagcataatccgggtgcaagcgcagcaccgtgttgtgttccgcaggcactggaaccgctgccgattgtttattatgttggtcgtaaaccgaaagttgaacagctgagcaatatgattgttcgtagctgtaaatgtagc

SEQ ID NO: 232 - protein, 112 aa, synthetic construct
ALDTNYCFSSTEKNCCVRQLYIDFRKDLGWKWIHEPKGYHANFCLGPCPYIWSLDTQYSKVLALYNQHNPGASAAPCCVPQALEPLPIVYYVGRKPKVEQLSNMIVRSCKCS

SEQ ID NO: 233 - DNA, 118 bp, synthetic construct
  source 1..118: mol_type = other DNA
ggggcctcgcttgggttattgctggtgcccggccgggcgcaatattcatgttgatgatttattatatatcgagtggtgtatttatttatattgtttgctccgttaccgttattaacag

SEQ ID NO: 234 - DNA, 52 bp, synthetic construct
  source 1..52: mol_type = other DNA
attggatccaattgacagctagctcagtcctaggtaccattggatccaatag

SEQ ID NO: 235 - DNA, 966 bp, synthetic construct
  source 1..966: mol_type = other DNA
ggggcctcgcttgggttattgctggtgcccggccgggcgcaatattcatgttgatgatttattatatatcgagtggtgtatttatttatattgtttgctccgttaccgttattaacagctgtcaccggatgtgctttccggtctgatgagtccgtgaggacgaaacagcctctacaaataattttgtttaatactagagaaagaggggaaatactagatgaagaaaaagatcattagcgcgatcctgatgagcaccgtgattctgagcgcggcggcgccgctgagcggtgtttatgcgagcccgggtcagggtacccaaagcgaaaacagctgcacccacttcccgggcaacctgccgaacatgctgcgtgacctgcgtgatgcgttcagccgtgtgaaaaccttcttccagatgaaagaccaactggataacctgctgctgaaggagagcctgctggaggacttcaaaggttacctgggctgccaggcgctgagcgaaatgatccaattttatctggaggaagtgatgccgcaggcggagaaccaagacccggatattaaggcgcacgttaacagcctgggcgagaacctgaaaaccctgcgtctgcgtctgcgtcgttgccaccgtttcctgccgtgcgagaacaaaagcaaggcggtggaacaggttaagaacgcgtttaacaaactgcaagagaagggcatctataaagcgatgagcgaattcgatatctttattaactacatcgaggcgtatatgaccatgaaaattcgtaactaggagctcgatagtgctagtgtagatcgctactagagccaggcatcaaataaaacgaaaggctcagtcgaaagactgggcctttcgttttatctgttgtttgtcggtgaacgctctctactagagtcacactggctcaccttcgggtgggcctttctgcgtttatatactagaagcggccgctgcag

SEQ ID NO: 236 - DNA, 900 bp, synthetic construct
  source 1..900: mol_type = other DNA
ggggcctcgcttgggttattgctggtgcccggccgggcgcaatattcatgttgatgatttattatatatcgagtggtgtatttatttatattgtttgctccgttaccgttattaacagctgtcaccggatgtgctttccggtctgatgagtccgtgaggacgaaacagcctctacaaataattttgtttaatactagagaaagaggggaaatactagatgaagaaaaagatcattagcgcgatcctgatgagcaccgtgattctgagcgcggcggcgccgctgagcggtgtttatgcgggtattacaatcccgcgtaatccgggttgtccgaatagtgaagataaaaattttccgcgtacagttatggttaatctgaatattcataaccgtaacacaaacaccaatccgaaacgtagtagcgattattataatcgtagcacaagcccgtggaatctgcatcgtaacgaagatccggaacgttatccaagcgttatctgggaagcaaaatgccgccatctgggttgtatcaatgcagatggtaacgttgattatcatatgaatagcgtgccgattcagcaggaaattctggttctgcgtcgtgaaccgccgcattgtccgaatagctttcgtctggaaaaaattctggttagcgttggttgtacctgtgttaccccgattgttcatcatgttgcacatcatcatcatcatcattaagagctcgatagtgctagtgtagatcgctactagagccaggcatcaaataaaacgaaaggctcagtcgaaagactgggcctttcgttttatctgttgtttgtcggtgaacgctctctactagagtcacactggctcaccttcgggtgggcctttctgcgtttatatactagaagcggccgctgcag

SEQ ID NO: 237 - DNA, 963 bp, synthetic construct
  source 1..963: mol_type = other DNA
ggggcctcgcttgggttattgctggtgcccggccgggcgcaatattcatgttgatgatttattatatatcgagtggtgtatttatttatattgtttgctccgttaccgttattaacagctgtcaccggatgtgctttccggtctgatgagtccgtgaggacgaaacagcctctacaaataattttgtttaatactagagaaagaggggaaatactagatgaagaaaaagatcattagcgcgatcctgatgagcaccgtgattctgagcgcggcggcgccgctgagcggtgtttatgcgctgcgtcgttgtctgattagcaccgatatgcatcatattgaagaaagctttcaggaaattaaacgtgccattcaggcaaaagatacctttccgaatgttaccattctgagcaccctggaaaccctgcagattatcaaaccactggatgtttgttgtgttaccaaaaatctgctggccttttatgttgatcgtgtttttaaagatcatcaggaaccgaatccgaaaattctgcgtaaaattagtagcattgccaatagctttctgtatatgcagaaaaccctgcgccagtgtcaggaacagcgtcagtgtcattgtcgtcaggaagcaaccaatgcaacccgtgtgattcatgataactatgatcagctggaagttcatgcagcagcgattaaaagcctgggtgaactggatgtgtttctggcatggattaataaaaatcatgaagtgatgtttagcgcacatcatcatcatcatcattaagagctcgatagtgctagtgtagatcgctactagagccaggcatcaaataaaacgaaaggctcagtcgaaagactgggcctttcgttttatctgttgtttgtcggtgaacgctctctactagagtcacactggctcaccttcgggtgggcctttctgcgtttatatactagaagcggccgctgcag

SEQ ID NO: 238 - DNA, 1986 bp, synthetic construct
  source 1..1986: mol_type = other DNA
ggggcctcgcttgggttattgctggtgcccggccgggcgcaatattcatgttgatgatttattatatatcgagtggtgtatttatttatattgtttgctccgttaccgttattaacagctgtcaccggatgtgctttccggtctgatgagtccgtgaggacgaaacagcctctacaaataattttgtttaatactagagaaagaggggaaatactagatgaagaaaaagatcattagcgcgatcctgatgagcaccgtgattctgagcgcggcggcgccgctgagcggtgtttatgcgatctgggaactgaaaaaggatgtttatgtggttgaactggattggtatccggatgcaccgggcgaaatggtggttctgacgtgtgatacgccggaagaagatggtattacctggacactggatcagagcagcgaagttctgggcagtggtaaaaccctgacgattcaggttaaagaatttggtgatgcaggtcagtatacctgtcataaaggtggtgaagttctgagccattccctgctgctgctgcataaaaaggaagatggtatctggagcaccgatattctgaaagatcagaaagaaccgaaaaacaaaacctttctgcgttgcgaagcgaaaaattattcaggccgttttacctgttggtggctgacgaccattagcacagatctgacctttagcgtgaaaagcagccgtggtagcagcgatccgcagggtgttacttgtggtgcagcaacgctgtctgcagaacgtgttcgtggtgataataaagaatatgaatatagcgtggaatgccaggaagattcagcatgtccggcagcagaagaaagcctgccgattgaagtgatggttgatgcagttcataaactgaaatatgaaaactataccagcagcttttttatccgtgatattattaaaccggaccctccgaaaaatctgcagctgaaacctctgaaaaatagtcgtcaggtggaagtgtcctgggaatatccggatacctggagcaccccacatagctattttagtctgaccttttgtgttcaggttcagggcaaatcaaaacgcgaaaaaaaagatcgtgtttttaccgataaaaccagcgcaaccgttatttgtcgtaaaaatgcaagcattagcgttcgtgcacaggatcgttattatagcagcagctggagcgaatgggcaagcgttccgtgtagcggtagcaccagcggtagcggtaaaccgggtagcggtgaaggtagcaccaaaggtcgtgcagttccgggtggtagcagcccggcatggacccagtgtcagcagctgagccagaaactgtgtaccctggcatggagcgcacatccgctggttggtcatatggatctgcgtgaagaaggtgatgaagaaaccaccaatgatgttccgcatattcagtgtggtgatggttgtgatccgcagggtctgcgtgataatagccagttttgtctgcagcgtattcatcagggtctgattttttatgaaaaactgctgggtagcgatatttttaccggtgaaccgagcctgctgccggatagcccggttggtcagctgcatgcaagcctgctgggtctgagccagctgctgcagccggaaggtcatcattgggaaacccagcagattccgagcctgagcccgagccagccgtggcagcgtctgctgctgcgttttaaaattctgcgtagcctgcaggcatttgttgcagttgcagcacgtgtttttgcacatggtgcagcaaccctgagcccgcatcatcatcatcatcattaagagctcgatagtgctagtgtagatcgctactagagccaggcatcaaataaaacgaaaggctcagtcgaaagactgggcctttcgttttatctgttgtttgtcggtgaacgctctctactagagtcacactggctcaccttcgggtgggcctttctgcgtttatatactagaagcggccgctgcag

SEQ ID NO: 239 - DNA, 1782 bp, synthetic construct
  source 1..1782: mol_type = other DNA
ggggcctcgcttgggttattgctggtgcccggccgggcgcaatattcatgttgatgatttattatatatcgagtggtgtatttatttatattgtttgctccgttaccgttattaacagctgtcaccggatgtgctttccggtctgatgagtccgtgaggacgaaacagcctctacaaataattttgtttaatactagagaaagaggggaaatactagatgaagaaaaagatcattagcgcgatcctgatgagcaccgtgattctgagcgcggcggcgccgctgagcggtgtttatgcgcgcaaaggtccgccggcagcactgaccctgccgcgtgttcagtgtcgtgcatcccgctatccgattgcagttgattgtagttggaccctgccgccggcaccgaattccacctcaccggttagctttattgctacctatcgtctgggtatggccgcacgtggtcattcatggccttgtctgcagcagaccccgaccagcacgagctgtaccatcaccgatgttcagctgttttctatggcaccgtatgttctgaatgttacggcagttcatccgtggggttcaagcagctcttttgttccatttattaccgaacatatcatcaaaccggaccctccggaaggtgttcgtctgagcccgctggcagaacgtcagctgcaggttcagtgggaaccgccaggttcatggccgtttcctgaaatttttagcctgaaatattggattcgttataaacgtcagggtgcggcccgttttcatcgtgttggtcctattgaagcaacctcatttattctgcgtgcggtccgtcctcgtgcccgttattatgttcaggtcgccgcacaggatctgaccgattatggtgaactgagcgattggtcactgccggcaaccgcgaccatgtccctgggtaaaggtggcggcggtagcggcggcggtggtagtggtggcggcggctctggcggcggcggttcccgtaacctgccggttgcgaccccggaccctggcatgtttccgtgtctgcatcattctcagaatctgctgcgtgcagtctctaatatgctgcagaaagcacgtcagaccctggaattttatccgtgtaccagtgaagaaatcgatcatgaagatattaccaaagataaaaccagcaccgtggaagcatgtctgccgctggaactgaccaaaaacgaaagctgtctgaacagccgcgaaaccagttttattacaaatggtagttgtctggcaagccgcaaaaccagctttatgatggcgctgtgtctgagctcaatttatgaagatctgaaaatgtatcaggtggaatttaaaaccatgaatgccaaactgctgatggaccctaaacgtcagatttttctggatcagaatatgctggcagttatcgatgaactgatgcaggcactgaactttaatagcgaaaccgttccgcagaaaagctccctggaagaaccggatttttataaaaccaaaatcaaactgtgcatcctgctgcatgcatttcgtattcgtgcagttaccattgatcgtgtgatgagctatctgaatgcaagccatcatcatcatcatcattaagagctcgatagtgctagtgtagatcgctactagagccaggcatcaaataaaacgaaaggctcagtcgaaagactgggcctttcgttttatctgttgtttgtcggtgaacgctctctactagagtcacactggctcaccttcgggtgggcctttctgcgtttatatactagaagcggccgctgcag

SEQ ID NO: 240 - DNA, 1023 bp, synthetic construct
  source 1..1023: mol_type = other DNA
ggggcctcgcttgggttattgctggtgcccggccgggcgcaatattcatgttgatgatttattatatatcgagtggtgtatttatttatattgtttgctccgttaccgttattaacagctgtcaccggatgtgctttccggtctgatgagtccgtgaggacgaaacagcctctacaaataattttgtttaatactagagaaagaggggaaatactagatgaagaaaaagatcattagcgcgatcctgatgagcaccgtgattctgagcgcggcggcgccgctgagcggtgtttatgcggttcataccagtccgaaagtgaaaaatctgaatccgaaaaagtttagcatccatgatcaggatcataaagttctggtactggatagcggtaatctgattgcagtgccggataaaaattatattcgtccggaaattttttttgccctggcaagcagcctgagttcagcctcagcggaaaaaggtagcccgattctgctgggtgttagtaaaggtgaattttgtctgtattgtgataaagataaaggccagagccatccgagtctgcagctgaaaaaggaaaaactgatgaaactggcagcacagaaagaaagcgctcgtcgtccgtttattttttatcgtgcacaggtgggtagctggaatatgctggaaagcgcagcccatccaggttggtttatttgcaccagctgcaattgtaatgaaccggtgggtgttaccgataaatttgaaaatcgtaaacatatcgaatttagctttcagccggtttgtaaagcagaaatgagcccgagcgaagttagtgatcatcatcatcatcatcattaagagctcgatagtgctagtgtagatcgctactagagccaggcatcaaataaaacgaaaggctcagtcgaaagactgggcctttcgttttatctgttgtttgtcggtgaacgctctctactagagtcacactggctcaccttcgggtgggcctttctgcgtttatatactagaagcggccgctgcag

SEQ ID NO: 241 - DNA, 840 bp, synthetic construct
  source 1..840: mol_type = other DNA
ggggcctcgcttgggttattgctggtgcccggccgggcgcaatattcatgttgatgatttattatatatcgagtggtgtatttatttatattgtttgctccgttaccgttattaacagctgtcaccggatgtgctttccggtctgatgagtccgtgaggacgaaacagcctctacaaataattttgtttaatactagagaaagaggggaaatactagatgaagaaaaagatcattagcgcgatcctgatgagcaccgtgattctgagcgcggcggcgccgctgagcggtgtttatgcggcactggataccaattattgtttttcaagcaccgaaaaaaattgttgtgttcgtcagctgtatattgattttcgtaaagatctgggttggaaatggattcatgaaccgaaaggttatcatgcaaatttttgtctgggtccgtgtccgtatatttggagcctggatacccagtatagcaaagttctggcactgtataatcagcataatccgggtgcaagcgcagcaccgtgttgtgttccgcaggcactggaaccgctgccgattgtttattatgttggtcgtaaaccgaaagttgaacagctgagcaatatgattgttcgtagctgtaaatgtagccatcatcatcatcatcattaagagctcgatagtgctagtgtagatcgctactagagccaggcatcaaataaaacgaaaggctcagtcgaaagactgggcctttcgttttatctgttgtttgtcggtgaacgctctctactagagtcacactggctcaccttcgggtgggcctttctgcgtttatatactagaagcggccgctgcag

SEQ ID NO: 242 - DNA, 115 bp, synthetic construct
  source 1..115: mol_type = other DNA
caaataaaacgaaaggctcagtcgaaagactgggcctttcgttttatctgttgtttgtcggtgaacgctctctactagagtcacactggctcaccttcgggtgggcctttctgcg

SEQ ID NO: 243 - DNA, 1253 bp, synthetic construct
  source 1..1253: mol_type = other DNA
atggcggcgcgccatcgaatggtgcaaaacctttcgcggtatggcatgatagcgcccggaagagagtcaattcatgggggttgaatatggaactgcgtgacctggatttaaacctgctggtggtgttcaaccagttgctggtcgacagacgcgtctctgtcactgcggagaacctgggcctgacccagcctgccgtgagcaatgcgctgaaacgcctgcgcacctcgctacaggacccactcttcgtgcgcacacatcagggaatggaacccacaccctatgccgcgcatctggccgagcacgtcacttcggccatgcacgcactgcgcaacgccctacagcaccatgaaagcttcgatccgctgaccagcgagcgtaccttcaccctggccatgaccgacattggcgagatctacttcatgccgcggctgatggatgcgctggctcaccaggcccccaattgcgtgatcagtacggtgcgcgacagttcgatgagcctgatgcaggccttgcagaacggaaccgtggacttggccgtgggcctgcttcccaatctgcaaactggcttctttcagcgccggctgctccagaatcactacgtgtgcctatgtcgcaaggaccatccagtcacccgcgaacccctgactctggagcgcttctgttcctacggccacgtgcgtgtcatcgccgctggcaccggccacggcgaggtggacacgtacatgacacgggtcggcatccggcgcgacatccgtctggaagtgccgcacttcgccgccgttggccacatcctccagcgcaccgatctgctcgccactgtgccgatatgtttagccgactgctgcgtagagcccttcggcctaagcgccttgccgcacccagtcgtcttgcctgaaatagccatcaacatgttctggcatgcgaagtaccacaaggacctagccaatatttggttgcggcaactgatgtttgacctgtttacggattgataaggatcctaattggtaacgaatcagacaattgacggctcgagggagtagcatagggtttgcagaatccctgcttcgtccatttgacaggcacattatgcatcgatgataagctgtcaaacatgagcagatcctctacgccggacgcatcgtggccggcatcaccggcgccacaggtgcggttgctggcgcctatatcgccgacatcaccgatggggaagatcgggctcgccacttcgggctcatgagcaaatattttatctg